European Patent Specification EP 3 426 686 B1, published October 8, 2025. Title: Humanized Anti-PACAP Antibodies and Uses Thereof. Applicant: Alder Biopharmaceuticals, Inc. Application TBA. The sequence listing filed with the application follows.

SEQUENCE LISTING (1600 sequences)

SEQ ID NO: 1-400 - skipped (400 entries)

SEQ ID NO: 401 - protein, 439 aa, Artificial
  Humanized antibody sequence
QSVEESGGRLVTPGTPLTLTCTVSGIDLNSYYMTWVRQAPGKGLEWIGFIDAGGDAYYASWAKGRFTISKTSTTVDLKITSPTTEDTATYFCARDLDLWGQGTLVTVSSASTKGPSVFPLAPSSKSTSGGTAALGCLVKDYFPEPVTVSWNSGALTSGVHTFPAVLQSSGLYSLSSVVTVPSSSLGTQTYICNVNHKPSNTKVDARVEPKSCDKTHTCPPCPAPELLGGPSVFLFPPKPKDTLMISRTPEVTCVVVDVSHEDPEVKFNWYVDGVEVHNAKTKPREEQYASTYRVVSVLTVLHQDWLNGKEYKCKVSNKALPAPIEKTISKAKGQPREPQVYTLPPSREEMTKNQVSLTCLVKGFYPSDIAVEWESNGQPENNYKTTPPVLDSDGSFFLYSKLTVDKSRWQQGNVFSCSVMHEALHNHYTQKSLSLSPGK

SEQ ID NO: 402 - protein, 109 aa, Artificial
  Humanized antibody sequence
QSVEESGGRLVTPGTPLTLTCTVSGIDLNSYYMTWVRQAPGKGLEWIGFIDAGGDAYYASWAKGRFTISKTSTTVDLKITSPTTEDTATYFCARDLDLWGQGTLVTVSS

SEQ ID NO: 403 - protein, 29 aa, Oryctolagus cuniculus
QSVEESGGRLVTPGTPLTLTCTVSGIDLN

SEQ ID NO: 404 - protein, 5 aa, Oryctolagus cuniculus
SYYMT

SEQ ID NO: 405 - protein, 14 aa, Oryctolagus cuniculus
WVRQAPGKGLEWIG

SEQ ID NO: 406 - protein, 16 aa, Oryctolagus cuniculus
FIDAGGDAYYASWAKG

SEQ ID NO: 407 - protein, 30 aa, Oryctolagus cuniculus
RFTISKTSTTVDLKITSPTTEDTATYFCAR

SEQ ID NO: 408 - protein, 4 aa, Oryctolagus cuniculus
DLDL

SEQ ID NO: 409 - protein, 11 aa, Artificial
  Humanized antibody sequence
WGQGTLVTVSS

SEQ ID NO: 410 - protein, 330 aa, Artificial
  Humanized antibody sequence
ASTKGPSVFPLAPSSKSTSGGTAALGCLVKDYFPEPVTVSWNSGALTSGVHTFPAVLQSSGLYSLSSVVTVPSSSLGTQTYICNVNHKPSNTKVDARVEPKSCDKTHTCPPCPAPELLGGPSVFLFPPKPKDTLMISRTPEVTCVVVDVSHEDPEVKFNWYVDGVEVHNAKTKPREEQYASTYRVVSVLTVLHQDWLNGKEYKCKVSNKALPAPIEKTISKAKGQPREPQVYTLPPSREEMTKNQVSLTCLVKGFYPSDIAVEWESNGQPENNYKTTPPVLDSDGSFFLYSKLTVDKSRWQQGNVFSCSVMHEALHNHYTQKSLSLSPGK

SEQ ID NO: 411 - DNA, 1317 bp, Artificial
  Humanized antibody sequence
cagtcggtggaggagtccgggggtcgcctggtcacgcctgggacacccctgacactcacctgcacagtctctggaatcgacctcaatagctactacatgacctgggtccgccaggctccagggaaggggctggaatggatcggattcattgatgctggtggtgacgcatactacgcgagctgggcgaaaggccgattcaccatctccaaaacctcgaccacggtggatctgaaaatcaccagtccgacaaccgaggacacggccacctatttctgtgccagagatcttgacttgtggggccagggcaccctggtcaccgtctcgagcgcctccaccaagggcccatcggtcttccccctggcaccctcctccaagagcacctctgggggcacagcggccctgggctgcctggtcaaggactacttccccgaaccggtgacggtgtcgtggaactcaggcgccctgaccagcggcgtgcacaccttcccggctgtcctacagtcctcaggactctactccctcagcagcgtggtgaccgtgccctccagcagcttgggcacccagacctacatctgcaacgtgaatcacaagcccagcaacaccaaggtggacgcgagagttgagcccaaatcttgtgacaaaactcacacatgcccaccgtgcccagcacctgaactcctggggggaccgtcagtcttcctcttccccccaaaacccaaggacaccctcatgatctcccggacccctgaggtcacatgcgtggtggtggacgtgagccacgaagaccctgaggtcaagttcaactggtacgtggacggcgtggaggtgcataatgccaagacaaagccgcgggaggagcagtacgccagcacgtaccgtgtggtcagcgtcctcaccgtcctgcaccaggactggctgaatggcaaggagtacaagtgcaaggtctccaacaaagccctcccagcccccatcgagaaaaccatctccaaagccaaagggcagccccgagaaccacaggtgtacaccctgcccccatcccgggaggagatgaccaagaaccaggtcagcctgacctgcctggtcaaaggcttctatcccagcgacatcgccgtggagtgggagagcaatgggcagccggagaacaactacaagaccacgcctcccgtgctggactccgacggctccttcttcctctacagcaagctcaccgtggacaagagcaggtggcagcaggggaacgtcttctcatgctccgtgatgcatgaggctctgcacaaccactacacgcagaagagcctctccctgtctccgggtaaa

SEQ ID NO: 412 - DNA, 327 bp, Artificial
  Humanized antibody sequence
cagtcggtggaggagtccgggggtcgcctggtcacgcctgggacacccctgacactcacctgcacagtctctggaatcgacctcaatagctactacatgacctgggtccgccaggctccagggaaggggctggaatggatcggattcattgatgctggtggtgacgcatactacgcgagctgggcgaaaggccgattcaccatctccaaaacctcgaccacggtggatctgaaaatcaccagtccgacaaccgaggacacggccacctatttctgtgccagagatcttgacttgtggggccagggcaccctggtcaccgtctcgagc

SEQ ID NO: 413 - DNA, 87 bp, Oryctolagus cuniculus
cagtcggtggaggagtccgggggtcgcctggtcacgcctgggacacccctgacactcacctgcacagtctctggaatcgacctcaat

SEQ ID NO: 414 - DNA, 15 bp, Oryctolagus cuniculus
agctactacatgacc

SEQ ID NO: 415 - DNA, 42 bp, Oryctolagus cuniculus
tgggtccgccaggctccagggaaggggctggaatggatcgga

SEQ ID NO: 416 - DNA, 48 bp, Oryctolagus cuniculus
ttcattgatgctggtggtgacgcatactacgcgagctgggcgaaaggc

SEQ ID NO: 417 - DNA, 90 bp, Oryctolagus cuniculus
cgattcaccatctccaaaacctcgaccacggtggatctgaaaatcaccagtccgacaaccgaggacacggccacctatttctgtgccaga

SEQ ID NO: 418 - DNA, 12 bp, Oryctolagus cuniculus
gatcttgacttg

SEQ ID NO: 419 - DNA, 33 bp, Artificial
  Humanized antibody sequence
tggggccagggcaccctggtcaccgtctcgagc

SEQ ID NO: 420 - DNA, 990 bp, Artificial
  Humanized antibody sequence
gcctccaccaagggcccatcggtcttccccctggcaccctcctccaagagcacctctgggggcacagcggccctgggctgcctggtcaaggactacttccccgaaccggtgacggtgtcgtggaactcaggcgccctgaccagcggcgtgcacaccttcccggctgtcctacagtcctcaggactctactccctcagcagcgtggtgaccgtgccctccagcagcttgggcacccagacctacatctgcaacgtgaatcacaagcccagcaacaccaaggtggacgcgagagttgagcccaaatcttgtgacaaaactcacacatgcccaccgtgcccagcacctgaactcctggggggaccgtcagtcttcctcttccccccaaaacccaaggacaccctcatgatctcccggacccctgaggtcacatgcgtggtggtggacgtgagccacgaagaccctgaggtcaagttcaactggtacgtggacggcgtggaggtgcataatgccaagacaaagccgcgggaggagcagtacgccagcacgtaccgtgtggtcagcgtcctcaccgtcctgcaccaggactggctgaatggcaaggagtacaagtgcaaggtctccaacaaagccctcccagcccccatcgagaaaaccatctccaaagccaaagggcagccccgagaaccacaggtgtacaccctgcccccatcccgggaggagatgaccaagaaccaggtcagcctgacctgcctggtcaaaggcttctatcccagcgacatcgccgtggagtgggagagcaatgggcagccggagaacaactacaagaccacgcctcccgtgctggactccgacggctccttcttcctctacagcaagctcaccgtggacaagagcaggtggcagcaggggaacgtcttctcatgctccgtgatgcatgaggctctgcacaaccactacacgcagaagagcctctccctgtctccgggtaaa

SEQ ID NO: 421 - protein, 216 aa, Artificial
  Humanized antibody sequence
AAVLTQTPSPVSAAVGGTVTINCQSSESVYGNYLAWFQQKPGQPPKLLIYEASKLESGVPSRFSGSGSGTQFTLTISDLQCDDAATYYCAGGDISEGVAFGGGTEVVVKRTVAAPSVFIFPPSDEQLKSGTASVVCLLNNFYPREAKVQWKVDNALQSGNSQESVTEQDSKDSTYSLSSTLTLSKADYEKHKVYACEVTHQGLSSPVTKSFNRGEC

SEQ ID NO: 422 - protein, 110 aa, Artificial
  Humanized antibody sequence
AAVLTQTPSPVSAAVGGTVTINCQSSESVYGNYLAWFQQKPGQPPKLLIYEASKLESGVPSRFSGSGSGTQFTLTISDLQCDDAATYYCAGGDISEGVAFGGGTEVVVKR

SEQ ID NO: 423 - protein, 23 aa, Oryctolagus cuniculus
AAVLTQTPSPVSAAVGGTVTINC

SEQ ID NO: 424 - protein, 12 aa, Oryctolagus cuniculus
QSSESVYGNYLA

SEQ ID NO: 425 - protein, 15 aa, Oryctolagus cuniculus
WFQQKPGQPPKLLIY

SEQ ID NO: 426 - protein, 7 aa, Oryctolagus cuniculus
EASKLES

SEQ ID NO: 427 - protein, 32 aa, Oryctolagus cuniculus
GVPSRFSGSGSGTQFTLTISDLQCDDAATYYC

SEQ ID NO: 428 - protein, 10 aa, Oryctolagus cuniculus
AGGDISEGVA

SEQ ID NO: 429 - protein, 11 aa, Artificial
  Humanized antibody sequence
FGGGTEVVVKR

SEQ ID NO: 430 - protein, 106 aa, Artificial
  Humanized antibody sequence
TVAAPSVFIFPPSDEQLKSGTASVVCLLNNFYPREAKVQWKVDNALQSGNSQESVTEQDSKDSTYSLSSTLTLSKADYEKHKVYACEVTHQGLSSPVTKSFNRGEC

SEQ ID NO: 431 - DNA, 648 bp, Artificial
  Humanized antibody sequence
gccgccgtgctgacccagactccatctcccgtgtctgcagctgtgggaggcacagtcaccatcaattgccagtccagtgagagtgtttacggtaactacttagcctggtttcagcagaaaccagggcagcctcccaagctcctgatctacgaagcatccaaactggaatctggggtcccatcgcggttcagcggcagtggatctgggacacagttcactctcaccatcagcgacttgcagtgtgacgatgctgccacttactactgtgcaggcggtgatattagtgaaggtgttgctttcggcggagggaccgaggtggtggtcaaacgtacggtagcggccccatctgtcttcatcttcccgccatctgatgagcagttgaaatctggaactgcctctgttgtgtgcctgctgaataacttctatcccagagaggccaaagtacagtggaaggtggataacgccctccaatcgggtaactcccaggagagtgtcacagagcaggacagcaaggacagcacctacagcctcagcagcaccctgacgctgagcaaagcagactacgagaaacacaaagtctacgcctgcgaagtcacccatcagggcctgagctcgcccgtcacaaagagcttcaacaggggagagtgt

SEQ ID NO: 432 - DNA, 330 bp, Artificial
  Humanized antibody sequence
gccgccgtgctgacccagactccatctcccgtgtctgcagctgtgggaggcacagtcaccatcaattgccagtccagtgagagtgtttacggtaactacttagcctggtttcagcagaaaccagggcagcctcccaagctcctgatctacgaagcatccaaactggaatctggggtcccatcgcggttcagcggcagtggatctgggacacagttcactctcaccatcagcgacttgcagtgtgacgatgctgccacttactactgtgcaggcggtgatattagtgaaggtgttgctttcggcggagggaccgaggtggtggtcaaacgt

SEQ ID NO: 433 - DNA, 69 bp, Oryctolagus cuniculus
gccgccgtgctgacccagactccatctcccgtgtctgcagctgtgggaggcacagtcaccatcaattgc

SEQ ID NO: 434 - DNA, 36 bp, Oryctolagus cuniculus
cagtccagtgagagtgtttacggtaactacttagcc

SEQ ID NO: 435 - DNA, 45 bp, Oryctolagus cuniculus
tggtttcagcagaaaccagggcagcctcccaagctcctgatctac

SEQ ID NO: 436 - DNA, 21 bp, Oryctolagus cuniculus
gaagcatccaaactggaatct

SEQ ID NO: 437 - DNA, 96 bp, Oryctolagus cuniculus
ggggtcccatcgcggttcagcggcagtggatctgggacacagttcactctcaccatcagcgacttgcagtgtgacgatgctgccacttactactgt

SEQ ID NO: 438 - DNA, 30 bp, Oryctolagus cuniculus
gcaggcggtgatattagtgaaggtgttgct

SEQ ID NO: 439 - DNA, 33 bp, Artificial
  Humanized antibody sequence
ttcggcggagggaccgaggtggtggtcaaacgt

SEQ ID NO: 440 - DNA, 318 bp, Artificial
  Humanized antibody sequence
acggtagcggccccatctgtcttcatcttcccgccatctgatgagcagttgaaatctggaactgcctctgttgtgtgcctgctgaataacttctatcccagagaggccaaagtacagtggaaggtggataacgccctccaatcgggtaactcccaggagagtgtcacagagcaggacagcaaggacagcacctacagcctcagcagcaccctgacgctgagcaaagcagactacgagaaacacaaagtctacgcctgcgaagtcacccatcagggcctgagctcgcccgtcacaaagagcttcaacaggggagagtgt

SEQ ID NO: 441 - protein, 439 aa, Artificial
  Humanized antibody sequence
QSVEESGGRLVTPGTPLTLTCTVSGIDLSSYYMSWVRQAPGKGLEWIGFIDTDGSAYYATWAKGRFTISKTSTTVDLKITSPTTEDTATYFCARDLDLWGPGTLVTVSSASTKGPSVFPLAPSSKSTSGGTAALGCLVKDYFPEPVTVSWNSGALTSGVHTFPAVLQSSGLYSLSSVVTVPSSSLGTQTYICNVNHKPSNTKVDKKVEPKSCDKTHTCPPCPAPELLGGPSVFLFPPKPKDTLMISRTPEVTCVVVDVSHEDPEVKFNWYVDGVEVHNAKTKPREEQYASTYRVVSVLTVLHQDWLNGKEYKCKVSNKALPAPIEKTISKAKGQPREPQVYTLPPSREEMTKNQVSLTCLVKGFYPSDIAVEWESNGQPENNYKTTPPVLDSDGSFFLYSKLTVDKSRWQQGNVFSCSVMHEALHNHYTQKSLSLSPGK

SEQ ID NO: 442 - protein, 109 aa, Artificial
  Humanized antibody sequence
QSVEESGGRLVTPGTPLTLTCTVSGIDLSSYYMSWVRQAPGKGLEWIGFIDTDGSAYYATWAKGRFTISKTSTTVDLKITSPTTEDTATYFCARDLDLWGPGTLVTVSS

SEQ ID NO: 443 - protein, 29 aa, Oryctolagus cuniculus
QSVEESGGRLVTPGTPLTLTCTVSGIDLS

SEQ ID NO: 444 - protein, 5 aa, Oryctolagus cuniculus
SYYMS

SEQ ID NO: 445 - protein, 14 aa, Oryctolagus cuniculus
WVRQAPGKGLEWIG

SEQ ID NO: 446 - protein, 16 aa, Oryctolagus cuniculus
FIDTDGSAYYATWAKG

SEQ ID NO: 447 - protein, 30 aa, Oryctolagus cuniculus; identical to SEQ ID NO: 407

SEQ ID NO: 448 - protein, 4 aa, Oryctolagus cuniculus
DLDL

SEQ ID NO: 449 - protein, 11 aa, Artificial
  Humanized antibody sequence
WGPGTLVTVSS

SEQ ID NO: 450 - protein, 330 aa, Artificial
  Humanized antibody sequence
ASTKGPSVFPLAPSSKSTSGGTAALGCLVKDYFPEPVTVSWNSGALTSGVHTFPAVLQSSGLYSLSSVVTVPSSSLGTQTYICNVNHKPSNTKVDKKVEPKSCDKTHTCPPCPAPELLGGPSVFLFPPKPKDTLMISRTPEVTCVVVDVSHEDPEVKFNWYVDGVEVHNAKTKPREEQYASTYRVVSVLTVLHQDWLNGKEYKCKVSNKALPAPIEKTISKAKGQPREPQVYTLPPSREEMTKNQVSLTCLVKGFYPSDIAVEWESNGQPENNYKTTPPVLDSDGSFFLYSKLTVDKSRWQQGNVFSCSVMHEALHNHYTQKSLSLSPGK

SEQ ID NO: 451 - DNA, 1317 bp, Artificial
  Humanized antibody sequence
cagtcggtggaggagtccgggggtcgcctggtcacgcctgggacacccctgacactcacctgcacagtctctggaatcgacctcagtagctactacatgagctgggtccgccaggctccagggaaggggctggaatggatcggattcattgatactgatggtagcgcatactacgcgacctgggcgaaaggccgattcaccatctccaaaacctcgaccacggtggatctgaaaatcaccagtccgacaaccgaggacacggccacctatttctgtgccagagatcttgacttgtggggcccgggcaccctcgtcaccgtctcgagcgcctccaccaagggcccatcggtcttccccctggcaccctcctccaagagcacctctgggggcacagcggccctgggctgcctggtcaaggactacttccccgaaccggtgacggtgtcgtggaactcaggcgccctgaccagcggcgtgcacaccttcccggctgtcctacagtcctcaggactctactccctcagcagcgtggtgaccgtgccctccagcagcttgggcacccagacctacatctgcaacgtgaatcacaagcccagcaacaccaaggtggacaagaaagttgagcccaaatcttgtgacaaaactcacacatgcccaccgtgcccagcacctgaactcctggggggaccgtcagtcttcctcttccccccaaaacccaaggacaccctcatgatctcccggacccctgaggtcacatgcgtggtggtggacgtgagccacgaagaccctgaggtcaagttcaactggtacgtggacggcgtggaggtgcataatgccaagacaaagccgcgggaggagcagtacgccagcacgtaccgtgtggtcagcgtcctcaccgtcctgcaccaggactggctgaatggcaaggagtacaagtgcaaggtctccaacaaagccctcccagcccccatcgagaaaaccatctccaaagccaaagggcagccccgagaaccacaggtgtacaccctgcccccatcccgggaggagatgaccaagaaccaggtcagcctgacctgcctggtcaaaggcttctatcccagcgacatcgccgtggagtgggagagcaatgggcagccggagaacaactacaagaccacgcctcccgtgctggactccgacggctccttcttcctctacagcaagctcaccgtggacaagagcaggtggcagcaggggaacgtcttctcatgctccgtgatgcatgaggctctgcacaaccactacacgcagaagagcctctccctgtctccgggtaaa

SEQ ID NO: 452 - DNA, 327 bp, Artificial
  Humanized antibody sequence
cagtcggtggaggagtccgggggtcgcctggtcacgcctgggacacccctgacactcacctgcacagtctctggaatcgacctcagtagctactacatgagctgggtccgccaggctccagggaaggggctggaatggatcggattcattgatactgatggtagcgcatactacgcgacctgggcgaaaggccgattcaccatctccaaaacctcgaccacggtggatctgaaaatcaccagtccgacaaccgaggacacggccacctatttctgtgccagagatcttgacttgtggggcccgggcaccctcgtcaccgtctcgagc

SEQ ID NO: 453 - DNA, 87 bp, Oryctolagus cuniculus
cagtcggtggaggagtccgggggtcgcctggtcacgcctgggacacccctgacactcacctgcacagtctctggaatcgacctcagt

SEQ ID NO: 454 - DNA, 15 bp, Oryctolagus cuniculus
agctactacatgagc

SEQ ID NO: 455 - DNA, 42 bp, Oryctolagus cuniculus; identical to SEQ ID NO: 415

SEQ ID NO: 456 - DNA, 48 bp, Oryctolagus cuniculus
ttcattgatactgatggtagcgcatactacgcgacctgggcgaaaggc

SEQ ID NO: 457 - DNA, 90 bp, Oryctolagus cuniculus; identical to SEQ ID NO: 417

SEQ ID NO: 458 - DNA, 12 bp, Oryctolagus cuniculus
gatcttgacttg

SEQ ID NO: 459 - DNA, 33 bp, Artificial
  Humanized antibody sequence
tggggcccgggcaccctcgtcaccgtctcgagc

SEQ ID NO: 460 - DNA, 990 bp, Artificial
  Humanized antibody sequence
gcctccaccaagggcccatcggtcttccccctggcaccctcctccaagagcacctctgggggcacagcggccctgggctgcctggtcaaggactacttccccgaaccggtgacggtgtcgtggaactcaggcgccctgaccagcggcgtgcacaccttcccggctgtcctacagtcctcaggactctactccctcagcagcgtggtgaccgtgccctccagcagcttgggcacccagacctacatctgcaacgtgaatcacaagcccagcaacaccaaggtggacaagaaagttgagcccaaatcttgtgacaaaactcacacatgcccaccgtgcccagcacctgaactcctggggggaccgtcagtcttcctcttccccccaaaacccaaggacaccctcatgatctcccggacccctgaggtcacatgcgtggtggtggacgtgagccacgaagaccctgaggtcaagttcaactggtacgtggacggcgtggaggtgcataatgccaagacaaagccgcgggaggagcagtacgccagcacgtaccgtgtggtcagcgtcctcaccgtcctgcaccaggactggctgaatggcaaggagtacaagtgcaaggtctccaacaaagccctcccagcccccatcgagaaaaccatctccaaagccaaagggcagccccgagaaccacaggtgtacaccctgcccccatcccgggaggagatgaccaagaaccaggtcagcctgacctgcctggtcaaaggcttctatcccagcgacatcgccgtggagtgggagagcaatgggcagccggagaacaactacaagaccacgcctcccgtgctggactccgacggctccttcttcctctacagcaagctcaccgtggacaagagcaggtggcagcaggggaacgtcttctcatgctccgtgatgcatgaggctctgcacaaccactacacgcagaagagcctctccctgtctccgggtaaa

SEQ ID NO: 461 - protein, 216 aa, Artificial
  Humanized antibody sequence
AAVLTQTPSPVSAAVGGTVSISCQSSESVYSNYLAWFQQKPGQPPKFLIYEASKLASGVPSRFKGSGSGTQFTLTISDVQCDDAGTYYCAGGYSSEGVAFGGGTEVVVKRTVAAPSVFIFPPSDEQLKSGTASVVCLLNNFYPREAKVQWKVDNALQSGNSQESVTEQDSKDSTYSLSSTLTLSKADYEKHKVYACEVTHQGLSSPVTKSFNRGEC

SEQ ID NO: 462 - protein, 110 aa, Artificial
  Humanized antibody sequence
AAVLTQTPSPVSAAVGGTVSISCQSSESVYSNYLAWFQQKPGQPPKFLIYEASKLASGVPSRFKGSGSGTQFTLTISDVQCDDAGTYYCAGGYSSEGVAFGGGTEVVVKR

SEQ ID NO: 463 - protein, 23 aa, Oryctolagus cuniculus
AAVLTQTPSPVSAAVGGTVSISC

SEQ ID NO: 464 - protein, 12 aa, Oryctolagus cuniculus
QSSESVYSNYLA

SEQ ID NO: 465 - protein, 15 aa, Oryctolagus cuniculus
WFQQKPGQPPKFLIY

SEQ ID NO: 466 - protein, 7 aa, Oryctolagus cuniculus
EASKLAS

SEQ ID NO: 467 - protein, 32 aa, Oryctolagus cuniculus
GVPSRFKGSGSGTQFTLTISDVQCDDAGTYYC

SEQ ID NO: 468 - protein, 10 aa, Oryctolagus cuniculus
AGGYSSEGVA

SEQ ID NO: 469 - protein, 11 aa, Artificial
  Humanized antibody sequence
FGGGTEVVVKR

SEQ ID NO: 470 - protein, 106 aa, Artificial; identical to SEQ ID NO: 430
  Humanized antibody sequence

SEQ ID NO: 471 - DNA, 648 bp, Artificial
  Humanized antibody sequence
gccgccgtgctgacccagactccatctcccgtgtctgcagctgtgggaggcacagtcagcatcagttgccagtccagtgagagtgtttatagtaactacttagcctggtttcagcagaaaccagggcagcctcctaagttcttgatctacgaagcatccaaactggcatctggggtcccatcgcggttcaaaggcagtggatctgggacacagttcactctcaccatcagcgacgtgcagtgtgacgatgctggcacttactactgtgcaggcggctatagtagtgaaggtgttgctttcggcggagggaccgaggtggtggtcaaacgtacggtagcggccccatctgtcttcatcttcccgccatctgatgagcagttgaaatctggaactgcctctgttgtgtgcctgctgaataacttctatcccagagaggccaaagtacagtggaaggtggataacgccctccaatcgggtaactcccaggagagtgtcacagagcaggacagcaaggacagcacctacagcctcagcagcaccctgacgctgagcaaagcagactacgagaaacacaaagtctacgcctgcgaagtcacccatcagggcctgagctcgcccgtcacaaagagcttcaacaggggagagtgt

SEQ ID NO: 472 - DNA, 330 bp, Artificial
  Humanized antibody sequence
gccgccgtgctgacccagactccatctcccgtgtctgcagctgtgggaggcacagtcagcatcagttgccagtccagtgagagtgtttatagtaactacttagcctggtttcagcagaaaccagggcagcctcctaagttcttgatctacgaagcatccaaactggcatctggggtcccatcgcggttcaaaggcagtggatctgggacacagttcactctcaccatcagcgacgtgcagtgtgacgatgctggcacttactactgtgcaggcggctatagtagtgaaggtgttgctttcggcggagggaccgaggtggtggtcaaacgt

SEQ ID NO: 473 - DNA, 69 bp, Oryctolagus cuniculus
gccgccgtgctgacccagactccatctcccgtgtctgcagctgtgggaggcacagtcagcatcagttgc

SEQ ID NO: 474 - DNA, 36 bp, Oryctolagus cuniculus
cagtccagtgagagtgtttatagtaactacttagcc

SEQ ID NO: 475 - DNA, 45 bp, Oryctolagus cuniculus
tggtttcagcagaaaccagggcagcctcctaagttcttgatctac

SEQ ID NO: 476 - DNA, 21 bp, Oryctolagus cuniculus
gaagcatccaaactggcatct

SEQ ID NO: 477 - DNA, 96 bp, Oryctolagus cuniculus
ggggtcccatcgcggttcaaaggcagtggatctgggacacagttcactctcaccatcagcgacgtgcagtgtgacgatgctggcacttactactgt

SEQ ID NO: 478 - DNA, 30 bp, Oryctolagus cuniculus
gcaggcggctatagtagtgaaggtgttgct

SEQ ID NO: 479 - DNA, 33 bp, Artificial; identical to SEQ ID NO: 439
  Humanized antibody sequence

SEQ ID NO: 480 - DNA, 318 bp, Artificial; identical to SEQ ID NO: 440
  Humanized antibody sequence

SEQ ID NO: 481-840 - skipped (360 entries)

SEQ ID NO: 841 - protein, 439 aa, Artificial
  Humanized antibody sequence
QSVEESGGRLVTPGTPLTLTCTVSGIDLSSYYMTWVRQAPGKGLEWVGFIDAGGSAYYATWAKGRFTISKASTTVDLKITSPTTEDTATYFCARDLDLWGPGTLVTVSSASTKGPSVFPLAPSSKSTSGGTAALGCLVKDYFPEPVTVSWNSGALTSGVHTFPAVLQSSGLYSLSSVVTVPSSSLGTQTYICNVNHKPSNTKVDKKVEPKSCDKTHTCPPCPAPELLGGPSVFLFPPKPKDTLMISRTPEVTCVVVDVSHEDPEVKFNWYVDGVEVHNAKTKPREEQYASTYRVVSVLTVLHQDWLNGKEYKCKVSNKALPAPIEKTISKAKGQPREPQVYTLPPSREEMTKNQVSLTCLVKGFYPSDIAVEWESNGQPENNYKTTPPVLDSDGSFFLYSKLTVDKSRWQQGNVFSCSVMHEALHNHYTQKSLSLSPGK

SEQ ID NO: 842 - protein, 109 aa, Artificial
  Humanized antibody sequence
QSVEESGGRLVTPGTPLTLTCTVSGIDLSSYYMTWVRQAPGKGLEWVGFIDAGGSAYYATWAKGRFTISKASTTVDLKITSPTTEDTATYFCARDLDLWGPGTLVTVSS

SEQ ID NO: 843 - protein, 29 aa, Oryctolagus cuniculus
QSVEESGGRLVTPGTPLTLTCTVSGIDLS

SEQ ID NO: 844 - protein, 5 aa, Oryctolagus cuniculus
SYYMT

SEQ ID NO: 845 - protein, 14 aa, Oryctolagus cuniculus
WVRQAPGKGLEWVG

SEQ ID NO: 846 - protein, 16 aa, Oryctolagus cuniculus
FIDAGGSAYYATWAKG

SEQ ID NO: 847 - protein, 30 aa, Oryctolagus cuniculus
RFTISKASTTVDLKITSPTTEDTATYFCAR

SEQ ID NO: 848 - protein, 4 aa, Oryctolagus cuniculus
DLDL

SEQ ID NO: 849 - protein, 11 aa, Artificial
  Humanized antibody sequence
WGPGTLVTVSS

SEQ ID NO: 850 - protein, 330 aa, Artificial; identical to SEQ ID NO: 450
  Humanized antibody sequence

SEQ ID NO: 851 - DNA, 1317 bp, Artificial
  Humanized antibody sequence
cagtcggtggaggagtccgggggtcgcctggtcacgcctgggacacccctgacactcacctgcacagtctctggaatcgacctcagtagctactacatgacctgggtccgccaggctccagggaaggggctggaatgggtcggattcattgatgctggtggtagcgcatactacgcgacctgggcaaaaggccgattcaccatctccaaagcctcgaccacggtggatctgaaaatcaccagtccgacaaccgaggacacggccacctatttctgtgccagagatcttgacttgtggggcccgggcaccctggtcaccgtctcgagcgcctccaccaagggcccatcggtcttccccctggcaccctcctccaagagcacctctgggggcacagcggccctgggctgcctggtcaaggactacttccccgaaccggtgacggtgtcgtggaactcaggcgccctgaccagcggcgtgcacaccttcccggctgtcctacagtcctcaggactctactccctcagcagcgtggtgaccgtgccctccagcagcttgggcacccagacctacatctgcaacgtgaatcacaagcccagcaacaccaaggtggacaagaaagttgagcccaaatcttgtgacaaaactcacacatgcccaccgtgcccagcacctgaactcctggggggaccgtcagtcttcctcttccccccaaaacccaaggacaccctcatgatctcccggacccctgaggtcacatgcgtggtggtggacgtgagccacgaagaccctgaggtcaagttcaactggtacgtggacggcgtggaggtgcataatgccaagacaaagccgcgggaggagcagtacgccagcacgtaccgtgtggtcagcgtcctcaccgtcctgcaccaggactggctgaatggcaaggagtacaagtgcaaggtctccaacaaagccctcccagcccccatcgagaaaaccatctccaaagccaaagggcagccccgagaaccacaggtgtacaccctgcccccatcccgggaggagatgaccaagaaccaggtcagcctgacctgcctggtcaaaggcttctatcccagcgacatcgccgtggagtgggagagcaatgggcagccggagaacaactacaagaccacgcctcccgtgctggactccgacggctccttcttcctctacagcaagctcaccgtggacaagagcaggtggcagcaggggaacgtcttctcatgctccgtgatgcatgaggctctgcacaaccactacacgcagaagagcctctccctgtctccgggtaaa

SEQ ID NO: 852 - DNA, 327 bp, Artificial
  Humanized antibody sequence
cagtcggtggaggagtccgggggtcgcctggtcacgcctgggacacccctgacactcacctgcacagtctctggaatcgacctcagtagctactacatgacctgggtccgccaggctccagggaaggggctggaatgggtcggattcattgatgctggtggtagcgcatactacgcgacctgggcaaaaggccgattcaccatctccaaagcctcgaccacggtggatctgaaaatcaccagtccgacaaccgaggacacggccacctatttctgtgccagagatcttgacttgtggggcccgggcaccctggtcaccgtctcgagc

SEQ ID NO: 853 - DNA, 87 bp, Oryctolagus cuniculus; identical to SEQ ID NO: 453

SEQ ID NO: 854 - DNA, 15 bp, Oryctolagus cuniculus
agctactacatgacc

SEQ ID NO: 855 - DNA, 42 bp, Oryctolagus cuniculus
tgggtccgccaggctccagggaaggggctggaatgggtcgga

SEQ ID NO: 856 - DNA, 48 bp, Oryctolagus cuniculus
ttcattgatgctggtggtagcgcatactacgcgacctgggcaaaaggc

SEQ ID NO: 857 - DNA, 90 bp, Oryctolagus cuniculus
cgattcaccatctccaaagcctcgaccacggtggatctgaaaatcaccagtccgacaaccgaggacacggccacctatttctgtgccaga

SEQ ID NO: 858 - DNA, 12 bp, Oryctolagus cuniculus
gatcttgacttg

SEQ ID NO: 859 - DNA, 33 bp, Artificial
  Humanized antibody sequence
tggggcccgggcaccctggtcaccgtctcgagc

SEQ ID NO: 860 - DNA, 990 bp, Artificial; identical to SEQ ID NO: 460
  Humanized antibody sequence

SEQ ID NO: 861 - protein, 216 aa, Artificial
  Humanized antibody sequence
AAVLTQTPSPVSAAVGGTVSISCKSSESVYGDYLAWFQQKPGQPPKQLIYDASTLASGVPSRFKGSGSGTQFTLTISGVQCDDAATYYCAGGYVSAGVAFGGGTEVVVKRTVAAPSVFIFPPSDEQLKSGTASVVCLLNNFYPREAKVQWKVDNALQSGNSQESVTEQDSKDSTYSLSSTLTLSKADYEKHKVYACEVTHQGLSSPVTKSFNRGEC

SEQ ID NO: 862 - protein, 110 aa, Artificial
  Humanized antibody sequence
AAVLTQTPSPVSAAVGGTVSISCKSSESVYGDYLAWFQQKPGQPPKQLIYDASTLASGVPSRFKGSGSGTQFTLTISGVQCDDAATYYCAGGYVSAGVAFGGGTEVVVKR

SEQ ID NO: 863 - protein, 23 aa, Oryctolagus cuniculus
AAVLTQTPSPVSAAVGGTVSISC

SEQ ID NO: 864 - protein, 12 aa, Oryctolagus cuniculus
KSSESVYGDYLA

SEQ ID NO: 865 - protein, 15 aa, Oryctolagus cuniculus
WFQQKPGQPPKQLIY

SEQ ID NO: 866 - protein, 7 aa, Oryctolagus cuniculus
DASTLAS

SEQ ID NO: 867 - protein, 32 aa, Oryctolagus cuniculus
GVPSRFKGSGSGTQFTLTISGVQCDDAATYYC

SEQ ID NO: 868 - protein, 10 aa, Oryctolagus cuniculus
AGGYVSAGVA

SEQ ID NO: 869 - protein, 11 aa, Artificial
  Humanized antibody sequence
FGGGTEVVVKR

SEQ ID NO: 870 - protein, 106 aa, Artificial; identical to SEQ ID NO: 430
  Humanized antibody sequence

SEQ ID NO: 871 - DNA, 648 bp, Artificial
  Humanized antibody sequence
gccgccgtgctgacccagactccatctcccgtgtctgcagctgtgggaggcacagtcagcatcagttgcaagtccagtgagagcgtttatggtgactacttagcctggtttcagcagaaaccagggcagcctcccaagcaactgatctatgatgcatccactctggcatctggggtcccatcgcggttcaaaggcagtggatctgggacacagttcactctcaccatcagcggcgtgcagtgtgacgatgctgccacttactactgtgcaggcggttatgttagtgcaggtgttgctttcggcggagggaccgaggtggtggtcaaacgtacggtagcggccccatctgtcttcatcttcccgccatctgatgagcagttgaaatctggaactgcctctgttgtgtgcctgctgaataacttctatcccagagaggccaaagtacagtggaaggtggataacgccctccaatcgggtaactcccaggagagtgtcacagagcaggacagcaaggacagcacctacagcctcagcagcaccctgacgctgagcaaagcagactacgagaaacacaaagtctacgcctgcgaagtcacccatcagggcctgagctcgcccgtcacaaagagcttcaacaggggagagtgt

SEQ ID NO: 872 - DNA, 330 bp, Artificial
  Humanized antibody sequence
gccgccgtgctgacccagactccatctcccgtgtctgcagctgtgggaggcacagtcagcatcagttgcaagtccagtgagagcgtttatggtgactacttagcctggtttcagcagaaaccagggcagcctcccaagcaactgatctatgatgcatccactctggcatctggggtcccatcgcggttcaaaggcagtggatctgggacacagttcactctcaccatcagcggcgtgcagtgtgacgatgctgccacttactactgtgcaggcggttatgttagtgcaggtgttgctttcggcggagggaccgaggtggtggtcaaacgt

SEQ ID NO: 873 - DNA, 69 bp, Oryctolagus cuniculus; identical to SEQ ID NO: 473

SEQ ID NO: 874 - DNA, 36 bp, Oryctolagus cuniculus
aagtccagtgagagcgtttatggtgactacttagcc

SEQ ID NO: 875 - DNA, 45 bp, Oryctolagus cuniculus
tggtttcagcagaaaccagggcagcctcccaagcaactgatctat

SEQ ID NO: 876 - DNA, 21 bp, Oryctolagus cuniculus
gatgcatccactctggcatct

SEQ ID NO: 877 - DNA, 96 bp, Oryctolagus cuniculus
ggggtcccatcgcggttcaaaggcagtggatctgggacacagttcactctcaccatcagcggcgtgcagtgtgacgatgctgccacttactactgt

SEQ ID NO: 878 - DNA, 30 bp, Oryctolagus cuniculus
gcaggcggttatgttagtgcaggtgttgct

SEQ ID NO: 879 - DNA, 33 bp, Artificial; identical to SEQ ID NO: 439
  Humanized antibody sequence

SEQ ID NO: 880 - DNA, 318 bp, Artificial; identical to SEQ ID NO: 440
  Humanized antibody sequence

SEQ ID NO: 881 - protein, 442 aa, Artificial
  Humanized antibody sequence
QEQLVESGGGLVQPEGSLTLTCTASGFDFSSNAMCWVRQAPGKGLEWIGSIYNADGKNYYAIWAKGRFTISRTSSTTVTLQMTSLTAADTATYFCARDFDLWGQGTLVTVSSASTKGPSVFPLAPSSKSTSGGTAALGCLVKDYFPEPVTVSWNSGALTSGVHTFPAVLQSSGLYSLSSVVTVPSSSLGTQTYICNVNHKPSNTKVDARVEPKSCDKTHTCPPCPAPELLGGPSVFLFPPKPKDTLMISRTPEVTCVVVDVSHEDPEVKFNWYVDGVEVHNAKTKPREEQYASTYRVVSVLTVLHQDWLNGKEYKCKVSNKALPAPIEKTISKAKGQPREPQVYTLPPSREEMTKNQVSLTCLVKGFYPSDIAVEWESNGQPENNYKTTPPVLDSDGSFFLYSKLTVDKSRWQQGNVFSCSVMHEALHNHYTQKSLSLSPGK

SEQ ID NO: 882 - protein, 112 aa, Artificial
  Humanized antibody sequence
QEQLVESGGGLVQPEGSLTLTCTASGFDFSSNAMCWVRQAPGKGLEWIGSIYNADGKNYYAIWAKGRFTISRTSSTTVTLQMTSLTAADTATYFCARDFDLWGQGTLVTVSS

SEQ ID NO: 883 - protein, 30 aa, Oryctolagus cuniculus
QEQLVESGGGLVQPEGSLTLTCTASGFDFS

SEQ ID NO: 884 - protein, 5 aa, Oryctolagus cuniculus
SNAMC

SEQ ID NO: 885 - protein, 14 aa, Oryctolagus cuniculus
WVRQAPGKGLEWIG

SEQ ID NO: 886 - protein, 17 aa, Oryctolagus cuniculus
SIYNADGKNYYAIWAKG

SEQ ID NO: 887 - protein, 31 aa, Oryctolagus cuniculus
RFTISRTSSTTVTLQMTSLTAADTATYFCAR

SEQ ID NO: 888 - protein, 4 aa, Oryctolagus cuniculus
DFDL

SEQ ID NO: 889 - protein, 11 aa, Artificial
  Humanized antibody sequence
WGQGTLVTVSS

SEQ ID NO: 890 - protein, 330 aa, Artificial; identical to SEQ ID NO: 410
  Humanized antibody sequence

SEQ ID NO: 891 - DNA, 1326 bp, Artificial
  Humanized antibody sequence
caggagcagctggtggagtccgggggaggcctggtccagcctgagggatccctgacactcacctgcacagcctctggattcgacttcagtagcaatgcaatgtgctgggtccgccaggctccagggaagggcctggagtggatcggatccatttataatgctgatggtaagaattattacgcgatttgggcgaaaggccgattcaccatctccagaacctcgtcgaccacggtgactctgcaaatgaccagtctgacagccgcggacacggccacctatttctgtgcgagagactttgacttgtggggccagggcaccctcgtcaccgtctcgagcgcctccaccaagggcccatcggtcttccccctggcaccctcctccaagagcacctctgggggcacagcggccctgggctgcctggtcaaggactacttccccgaaccggtgacggtgtcgtggaactcaggcgccctgaccagcggcgtgcacaccttcccggctgtcctacagtcctcaggactctactccctcagcagcgtggtgaccgtgccctccagcagcttgggcacccagacctacatctgcaacgtgaatcacaagcccagcaacaccaaggtggacgcgagagttgagcccaaatcttgtgacaaaactcacacatgcccaccgtgcccagcacctgaactcctggggggaccgtcagtcttcctcttccccccaaaacccaaggacaccctcatgatctcccggacccctgaggtcacatgcgtggtggtggacgtgagccacgaagaccctgaggtcaagttcaactggtacgtggacggcgtggaggtgcataatgccaagacaaagccgcgggaggagcagtacgccagcacgtaccgtgtggtcagcgtcctcaccgtcctgcaccaggactggctgaatggcaaggagtacaagtgcaaggtctccaacaaagccctcccagcccccatcgagaaaaccatctccaaagccaaagggcagccccgagaaccacaggtgtacaccctgcccccatcccgggaggagatgaccaagaaccaggtcagcctgacctgcctggtcaaaggcttctatcccagcgacatcgccgtggagtgggagagcaatgggcagccggagaacaactacaagaccacgcctcccgtgctggactccgacggctccttcttcctctacagcaagctcaccgtggacaagagcaggtggcagcaggggaacgtcttctcatgctccgtgatgcatgaggctctgcacaaccactacacgcagaagagcctctccctgtctccgggtaaa

SEQ ID NO: 892 - DNA, 336 bp, Artificial
  Humanized antibody sequence
caggagcagctggtggagtccgggggaggcctggtccagcctgagggatccctgacactcacctgcacagcctctggattcgacttcagtagcaatgcaatgtgctgggtccgccaggctccagggaagggcctggagtggatcggatccatttataatgctgatggtaagaattattacgcgatttgggcgaaaggccgattcaccatctccagaacctcgtcgaccacggtgactctgcaaatgaccagtctgacagccgcggacacggccacctatttctgtgcgagagactttgacttgtggggccagggcaccctcgtcaccgtctcgagc

SEQ ID NO: 893 - DNA, 90 bp, Oryctolagus cuniculus
caggagcagctggtggagtccgggggaggcctggtccagcctgagggatccctgacactcacctgcacagcctctggattcgacttcagt

SEQ ID NO: 894 - DNA, 15 bp, Oryctolagus cuniculus
agcaatgcaatgtgc

SEQ ID NO: 895 - DNA, 42 bp, Oryctolagus cuniculus
tgggtccgccaggctccagggaagggcctggagtggatcgga

SEQ ID NO: 896 - DNA, 51 bp, Oryctolagus cuniculus
tccatttataatgctgatggtaagaattattacgcgatttgggcgaaaggc

SEQ ID NO: 897 - DNA, 93 bp, Oryctolagus cuniculus
cgattcaccatctccagaacctcgtcgaccacggtgactctgcaaatgaccagtctgacagccgcggacacggccacctatttctgtgcgaga

SEQ ID NO: 898 - DNA, 12 bp, Oryctolagus cuniculus
gactttgacttg

SEQ ID NO: 899 - DNA, 33 bp, Artificial
  Humanized antibody sequence
tggggccagggcaccctcgtcaccgtctcgagc

SEQ ID NO: 900 - DNA, 990 bp, Artificial; identical to SEQ ID NO: 420
  Humanized antibody sequence

SEQ ID NO: 901 - protein, 219 aa, Artificial
  Humanized antibody sequence
AAVLTQTPSPVSAAVGGTVTINCQSSQSVYDNDWLAWFQQKPGQPPKLLIYLTSTLASGVPSRFSGSGSGTQFTLTISGVQCDDAATYYCLGGYDEDGDTHVFGGGTEVVVKRTVAAPSVFIFPPSDEQLKSGTASVVCLLNNFYPREAKVQWKVDNALQSGNSQESVTEQDSKDSTYSLSSTLTLSKADYEKHKVYACEVTHQGLSSPVTKSFNRGEC

SEQ ID NO: 902 - protein, 113 aa, Artificial
  Humanized antibody sequence
AAVLTQTPSPVSAAVGGTVTINCQSSQSVYDNDWLAWFQQKPGQPPKLLIYLTSTLASGVPSRFSGSGSGTQFTLTISGVQCDDAATYYCLGGYDEDGDTHVFGGGTEVVVKR

SEQ ID NO: 903 - protein, 23 aa, Oryctolagus cuniculus
AAVLTQTPSPVSAAVGGTVTINC

SEQ ID NO: 904 - protein, 13 aa, Oryctolagus cuniculus
QSSQSVYDNDWLA

SEQ ID NO: 905 - protein, 15 aa, Oryctolagus cuniculus
WFQQKPGQPPKLLIY

SEQ ID NO: 906 - protein, 7 aa, Oryctolagus cuniculus
LTSTLAS

SEQ ID NO: 907 - protein, 32 aa, Oryctolagus cuniculus
GVPSRFSGSGSGTQFTLTISGVQCDDAATYYC

SEQ ID NO: 908 - protein, 12 aa, Oryctolagus cuniculus
LGGYDEDGDTHV

SEQ ID NO: 909 - protein, 11 aa, Artificial
  Humanized antibody sequence
FGGGTEVVVKR

SEQ ID NO: 910 - protein, 106 aa, Artificial; identical to SEQ ID NO: 430
  Humanized antibody sequence

SEQ ID NO: 911 - DNA, 657 bp, Artificial
  Humanized antibody sequence
gcagccgtgctgacccagacaccatcgcccgtgtctgcagctgtgggaggcacagtcaccatcaattgccagtccagtcagagtgtttatgataacgactggttagcctggttccagcagaaaccagggcagcctcccaagctcctgatctatctgacatccactctggcatctggagtcccatcgcggttcagcggcagtggatctgggacacagttcactctcaccatcagtggtgtgcagtgtgacgatgctgccacttactactgtctaggcggctatgatgaagatggtgatacgcatgttttcggcggagggaccgaggtggtggtcaaacgtacggtagcggccccatctgtcttcatcttcccgccatctgatgagcagttgaaatctggaactgcctctgttgtgtgcctgctgaataacttctatcccagagaggccaaagtacagtggaaggtggataacgccctccaatcgggtaactcccaggagagtgtcacagagcaggacagcaaggacagcacctacagcctcagcagcaccctgacgctgagcaaagcagactacgagaaacacaaagtctacgcctgcgaagtcacccatcagggcctgagctcgcccgtcacaaagagcttcaacaggggagagtgt

SEQ ID NO: 912 - DNA, 339 bp, Artificial
  Humanized antibody sequence
gcagccgtgctgacccagacaccatcgcccgtgtctgcagctgtgggaggcacagtcaccatcaattgccagtccagtcagagtgtttatgataacgactggttagcctggttccagcagaaaccagggcagcctcccaagctcctgatctatctgacatccactctggcatctggagtcccatcgcggttcagcggcagtggatctgggacacagttcactctcaccatcagtggtgtgcagtgtgacgatgctgccacttactactgtctaggcggctatgatgaagatggtgatacgcatgttttcggcggagggaccgaggtggtggtcaaacgt

SEQ ID NO: 913 - DNA, 69 bp, Oryctolagus cuniculus
gcagccgtgctgacccagacaccatcgcccgtgtctgcagctgtgggaggcacagtcaccatcaattgc

SEQ ID NO: 914 - DNA, 39 bp, Oryctolagus cuniculus
cagtccagtcagagtgtttatgataacgactggttagcc

SEQ ID NO: 915 - DNA, 45 bp, Oryctolagus cuniculus
tggttccagcagaaaccagggcagcctcccaagctcctgatctat

SEQ ID NO: 916 - DNA, 21 bp, Oryctolagus cuniculus
ctgacatccactctggcatct

SEQ ID NO: 917 - DNA, 96 bp, Oryctolagus cuniculus
ggagtcccatcgcggttcagcggcagtggatctgggacacagttcactctcaccatcagtggtgtgcagtgtgacgatgctgccacttactactgt

SEQ ID NO: 918 - DNA, 36 bp, Oryctolagus cuniculus
ctaggcggctatgatgaagatggtgatacgcatgtt

SEQ ID NO: 919 - DNA, 33 bp, Artificial; identical to SEQ ID NO: 439
  Humanized antibody sequence

SEQ ID NO: 920 - DNA, 318 bp, Artificial; identical to SEQ ID NO: 440
  Humanized antibody sequence

SEQ ID NO: 921 - protein, 447 aa, Artificial
  Humanized antibody sequence
QSVEESGGRLVTPGTPLTLTCTVSGFSLNNYAMSWVRQAPGKGLEWIGIMGVNDITYYASWAKGRFTISKTSTTVDLKMTSLTTEDTATYFCTREIRDDGDSSDKLWGPGTLVTVSSASTKGPSVFPLAPSSKSTSGGTAALGCLVKDYFPEPVTVSWNSGALTSGVHTFPAVLQSSGLYSLSSVVTVPSSSLGTQTYICNVNHKPSNTKVDARVEPKSCDKTHTCPPCPAPELLGGPSVFLFPPKPKDTLMISRTPEVTCVVVDVSHEDPEVKFNWYVDGVEVHNAKTKPREEQYASTYRVVSVLTVLHQDWLNGKEYKCKVSNKALPAPIEKTISKAKGQPREPQVYTLPPSREEMTKNQVSLTCLVKGFYPSDIAVEWESNGQPENNYKTTPPVLDSDGSFFLYSKLTVDKSRWQQGNVFSCSVMHEALHNHYTQKSLSLSPGK

SEQ ID NO: 922 - protein, 117 aa, Artificial
  Humanized antibody sequence
QSVEESGGRLVTPGTPLTLTCTVSGFSLNNYAMSWVRQAPGKGLEWIGIMGVNDITYYASWAKGRFTISKTSTTVDLKMTSLTTEDTATYFCTREIRDDGDSSDKLWGPGTLVTVSS

SEQ ID NO: 923 - protein, 29 aa, Oryctolagus cuniculus
QSVEESGGRLVTPGTPLTLTCTVSGFSLN

SEQ ID NO: 924 - protein, 5 aa, Oryctolagus cuniculus
NYAMS

SEQ ID NO: 925 - protein, 14 aa, Oryctolagus cuniculus
WVRQAPGKGLEWIG

SEQ ID NO: 926 - protein, 16 aa, Oryctolagus cuniculus
IMGVNDITYYASWAKG

SEQ ID NO: 927 - protein, 30 aa, Oryctolagus cuniculus
RFTISKTSTTVDLKMTSLTTEDTATYFCTR

SEQ ID NO: 928 - protein, 12 aa, Oryctolagus cuniculus
EIRDDGDSSDKL

SEQ ID NO: 929 - protein, 11 aa, Artificial
  Humanized antibody sequence
WGPGTLVTVSS

SEQ ID NO: 930 - protein, 330 aa, Artificial; identical to SEQ ID NO: 410
  Humanized antibody sequence

SEQ ID NO: 931 - DNA, 1341 bp, Artificial
  Humanized antibody sequence
cagtcggtggaggagtccgggggtcgcctggtcacgcctgggacacccctgacactcacctgcaccgtctctggattctccctcaataactatgcaatgagctgggtccgccaggctccagggaaggggctggaatggatcggaatcatgggtgttaatgatatcacatactacgcgagctgggcgaaaggccgattcaccatctccaaaacctcgaccacggtggatctgaaaatgaccagtctgacaaccgaggacacggccacctatttctgtactagagagatccgtgatgatggtgatagttctgataagttgtggggcccgggcaccctcgtcaccgtctcgagcgcctccaccaagggcccatcggtcttccccctggcaccctcctccaagagcacctctgggggcacagcggccctgggctgcctggtcaaggactacttccccgaaccggtgacggtgtcgtggaactcaggcgccctgaccagcggcgtgcacaccttcccggctgtcctacagtcctcaggactctactccctcagcagcgtggtgaccgtgccctccagcagcttgggcacccagacctacatctgcaacgtgaatcacaagcccagcaacaccaaggtggacgcgagagttgagcccaaatcttgtgacaaaactcacacatgcccaccgtgcccagcacctgaactcctggggggaccgtcagtcttcctcttccccccaaaacccaaggacaccctcatgatctcccggacccctgaggtcacatgcgtggtggtggacgtgagccacgaagaccctgaggtcaagttcaactggtacgtggacggcgtggaggtgcataatgccaagacaaagccgcgggaggagcagtacgccagcacgtaccgtgtggtcagcgtcctcaccgtcctgcaccaggactggctgaatggcaaggagtacaagtgcaaggtctccaacaaagccctcccagcccccatcgagaaaaccatctccaaagccaaagggcagccccgagaaccacaggtgtacaccctgcccccatcccgggaggagatgaccaagaaccaggtcagcctgacctgcctggtcaaaggcttctatcccagcgacatcgccgtggagtgggagagcaatgggcagccggagaacaactacaagaccacgcctcccgtgctggactccgacggctccttcttcctctacagcaagctcaccgtggacaagagcaggtggcagcaggggaacgtcttctcatgctccgtgatgcatgaggctctgcacaaccactacacgcagaagagcctctccctgtctccgggtaaa

SEQ ID NO: 932 - DNA, 351 bp, Artificial
  Humanized antibody sequence
cagtcggtggaggagtccgggggtcgcctggtcacgcctgggacacccctgacactcacctgcaccgtctctggattctccctcaataactatgcaatgagctgggtccgccaggctccagggaaggggctggaatggatcggaatcatgggtgttaatgatatcacatactacgcgagctgggcgaaaggccgattcaccatctccaaaacctcgaccacggtggatctgaaaatgaccagtctgacaaccgaggacacggccacctatttctgtactagagagatccgtgatgatggtgatagttctgataagttgtggggcccgggcaccctcgtcaccgtctcgagc

SEQ ID NO: 933 - DNA, 87 bp, Oryctolagus cuniculus
cagtcggtggaggagtccgggggtcgcctggtcacgcctgggacacccctgacactcacctgcaccgtctctggattctccctcaat

SEQ ID NO: 934 - DNA, 15 bp, Oryctolagus cuniculus
aactatgcaatgagc

SEQ ID NO: 935 - DNA, 42 bp, Oryctolagus cuniculus; identical to SEQ ID NO: 415

SEQ ID NO: 936 - DNA, 48 bp, Oryctolagus cuniculus
atcatgggtgttaatgatatcacatactacgcgagctgggcgaaaggc

SEQ ID NO: 937 - DNA, 90 bp, Oryctolagus cuniculus
cgattcaccatctccaaaacctcgaccacggtggatctgaaaatgaccagtctgacaaccgaggacacggccacctatttctgtactaga

SEQ ID NO: 938 - DNA, 36 bp, Oryctolagus cuniculus
gagatccgtgatgatggtgatagttctgataagttg

SEQ ID NO: 939 - DNA, 33 bp, Artificial; identical to SEQ ID NO: 459
  Humanized antibody sequence

SEQ ID NO: 940 - DNA, 990 bp, Artificial; identical to SEQ ID NO: 420
  Humanized antibody sequence

SEQ ID NO: 941 - protein, 219 aa, Artificial
  Humanized antibody sequence
AIKMTQTPSSVSAAVGGTVTINCQASEDIYTNLAWYQQKPGQPPNLLIYDASDLASGVPSRFSGSGDGTQFTLTISAVQCEDAATYYCQGVAWSSNTGYGSAFGGGTEVVVKRTVAAPSVFIFPPSDEQLKSGTASVVCLLNNFYPREAKVQWKVDNALQSGNSQESVTEQDSKDSTYSLSSTLTLSKADYEKHKVYACEVTHQGLSSPVTKSFNRGEC

SEQ ID NO: 942 - protein, 113 aa, Artificial
  Humanized antibody sequence
AIKMTQTPSSVSAAVGGTVTINCQASEDIYTNLAWYQQKPGQPPNLLIYDASDLASGVPSRFSGSGDGTQFTLTISAVQCEDAATYYCQGVAWSSNTGYGSAFGGGTEVVVKR

SEQ ID NO: 943 - protein, 23 aa, Oryctolagus cuniculus
AIKMTQTPSSVSAAVGGTVTINC

SEQ ID NO: 944 - protein, 11 aa, Oryctolagus cuniculus
QASEDIYTNLA

SEQ ID NO: 945 - protein, 15 aa, Oryctolagus cuniculus
WYQQKPGQPPNLLIY

SEQ ID NO: 946 - protein, 7 aa, Oryctolagus cuniculus
DASDLAS

SEQ ID NO: 947 - protein, 32 aa, Oryctolagus cuniculus
GVPSRFSGSGDGTQFTLTISAVQCEDAATYYC

SEQ ID NO: 948 - protein, 14 aa, Oryctolagus cuniculus
QGVAWSSNTGYGSA

SEQ ID NO: 949 - protein, 11 aa, Artificial
  Humanized antibody sequence
FGGGTEVVVKR

SEQ ID NO: 950 - protein, 106 aa, Artificial; identical to SEQ ID NO: 430
  Humanized antibody sequence

SEQ ID NO: 951 - DNA, 657 bp, Artificial
  Humanized antibody sequence
gccatcaaaatgacccagactccatcctccgtgtctgcagctgtgggaggcacagtcaccatcaattgccaggccagtgaggacatttacaccaatttagcctggtatcagcagaaaccagggcagcctcccaacctcctgatctatgatgcatccgatctggcatctggggtcccgtcgcggttcagcggcagtggagatgggacacagttcactctcaccatcagcgccgtgcagtgtgaagatgctgccacttactactgtcaaggtgttgcttggagtagtaatactggttatggttccgctttcggcggagggaccgaggtggtggtcaaacgtacggtagcggccccatctgtcttcatcttcccgccatctgatgagcagttgaaatctggaactgcctctgttgtgtgcctgctgaataacttctatcccagagaggccaaagtacagtggaaggtggataacgccctccaatcgggtaactcccaggagagtgtcacagagcaggacagcaaggacagcacctacagcctcagcagcaccctgacgctgagcaaagcagactacgagaaacacaaagtctacgcctgcgaagtcacccatcagggcctgagctcgcccgtcacaaagagcttcaacaggggagagtgt

SEQ ID NO: 952 - DNA, 339 bp, Artificial
  Humanized antibody sequence
gccatcaaaatgacccagactccatcctccgtgtctgcagctgtgggaggcacagtcaccatcaattgccaggccagtgaggacatttacaccaatttagcctggtatcagcagaaaccagggcagcctcccaacctcctgatctatgatgcatccgatctggcatctggggtcccgtcgcggttcagcggcagtggagatgggacacagttcactctcaccatcagcgccgtgcagtgtgaagatgctgccacttactactgtcaaggtgttgcttggagtagtaatactggttatggttccgctttcggcggagggaccgaggtggtggtcaaacgt

SEQ ID NO: 953 - DNA, 69 bp, Oryctolagus cuniculus
gccatcaaaatgacccagactccatcctccgtgtctgcagctgtgggaggcacagtcaccatcaattgc

SEQ ID NO: 954 - DNA, 33 bp, Oryctolagus cuniculus
caggccagtgaggacatttacaccaatttagcc

SEQ ID NO: 955 - DNA, 45 bp, Oryctolagus cuniculus
tggtatcagcagaaaccagggcagcctcccaacctcctgatctat

SEQ ID NO: 956 - DNA, 21 bp, Oryctolagus cuniculus
gatgcatccgatctggcatct

SEQ ID NO: 957 - DNA, 96 bp, Oryctolagus cuniculus
ggggtcccgtcgcggttcagcggcagtggagatgggacacagttcactctcaccatcagcgccgtgcagtgtgaagatgctgccacttactactgt

SEQ ID NO: 958 - DNA, 42 bp, Oryctolagus cuniculus
caaggtgttgcttggagtagtaatactggttatggttccgct

SEQ ID NO: 959 - DNA, 33 bp, Artificial; identical to SEQ ID NO: 439
  Humanized antibody sequence

SEQ ID NO: 960 - DNA, 318 bp, Artificial; identical to SEQ ID NO: 440
  Humanized antibody sequence

SEQ ID NO: 961 - protein, 442 aa, Artificial
  Humanized antibody sequence
EVQLVESGGGLVQPGGSLRLSCAASGIDLNSYYMTWVRQAPGKGLEWIGFIDAGGDAYYASWAKGRFTISRDNSKNTVYLQMNSLRAEDTAVYFCARDLDLWGQGTLVTVSSASTKGPSVFPLAPSSKSTSGGTAALGCLVKDYFPEPVTVSWNSGALTSGVHTFPAVLQSSGLYSLSSVVTVPSSSLGTQTYICNVNHKPSNTKVDKKVEPKSCDKTHTCPPCPAPELLGGPSVFLFPPKPKDTLMISRTPEVTCVVVDVSHEDPEVKFNWYVDGVEVHNAKTKPREEQYASTYRVVSVLTVLHQDWLNGKEYKCKVSNKALPAPIEKTISKAKGQPREPQVYTLPPSREEMTKNQVSLTCLVKGFYPSDIAVEWESNGQPENNYKTTPPVLDSDGSFFLYSKLTVDKSRWQQGNVFSCSVMHEALHNHYTQKSLSLSPGK

SEQ ID NO: 962 - protein, 112 aa, Artificial
  Humanized antibody sequence
EVQLVESGGGLVQPGGSLRLSCAASGIDLNSYYMTWVRQAPGKGLEWIGFIDAGGDAYYASWAKGRFTISRDNSKNTVYLQMNSLRAEDTAVYFCARDLDLWGQGTLVTVSS

SEQ ID NO: 963 - protein, 30 aa, Artificial
  Humanized antibody sequence
EVQLVESGGGLVQPGGSLRLSCAASGIDLN

SEQ ID NO: 964 - protein, 5 aa, Oryctolagus cuniculus
SYYMT

SEQ ID NO: 965 - protein, 14 aa, Artificial
  Humanized antibody sequence
WVRQAPGKGLEWIG

SEQ ID NO: 966 - protein, 16 aa, Oryctolagus cuniculus
FIDAGGDAYYASWAKG

SEQ ID NO: 967 - protein, 32 aa, Artificial
  Humanized antibody sequence
RFTISRDNSKNTVYLQMNSLRAEDTAVYFCAR

SEQ ID NO: 968 - protein, 4 aa, Oryctolagus cuniculus
DLDL

SEQ ID NO: 969 - protein, 11 aa, Artificial
  Humanized antibody sequence
WGQGTLVTVSS

SEQ ID NO: 970 - protein, 330 aa, Artificial; identical to SEQ ID NO: 450
  Humanized antibody sequence

SEQ ID NO: 971 - DNA, 1326 bp, Artificial
  Humanized antibody sequence
gaggtgcagcttgtggagtctgggggaggcttggtccagcctggggggtccctgagactctcctgtgcagcctctggaatcgacctcaatagctactacatgacctgggtccgtcaggctccagggaaggggctggagtggatcggattcattgatgctggtggtgacgcatactacgcgagctgggcgaaaggccgattcaccatctccagagacaattccaagaacaccgtgtatcttcaaatgaacagcctgagagctgaggacactgctgtgtatttctgtgctagagatcttgacttgtggggccaagggaccctcgtcaccgtctcgagcgcctccaccaagggcccatcggtcttccccctggcaccctcctccaagagcacctctgggggcacagcggccctgggctgcctggtcaaggactacttccccgaaccggtgacggtgtcgtggaactcaggcgccctgaccagcggcgtgcacaccttcccggctgtcctacagtcctcaggactctactccctcagcagcgtggtgaccgtgccctccagcagcttgggcacccagacctacatctgcaacgtgaatcacaagcccagcaacaccaaggtggacaagaaagttgagcccaaatcttgtgacaaaactcacacatgcccaccgtgcccagcacctgaactcctggggggaccgtcagtcttcctcttccccccaaaacccaaggacaccctcatgatctcccggacccctgaggtcacatgcgtggtggtggacgtgagccacgaagaccctgaggtcaagttcaactggtacgtggacggcgtggaggtgcataatgccaagacaaagccgcgggaggagcagtacgccagcacgtaccgtgtggtcagcgtcctcaccgtcctgcaccaggactggctgaatggcaaggagtacaagtgcaaggtctccaacaaagccctcccagcccccatcgagaaaaccatctccaaagccaaagggcagccccgagaaccacaggtgtacaccctgcccccatcccgggaggagatgaccaagaaccaggtcagcctgacctgcctggtcaaaggcttctatcccagcgacatcgccgtggagtgggagagcaatgggcagccggagaacaactacaagaccacgcctcccgtgctggactccgacggctccttcttcctctacagcaagctcaccgtggacaagagcaggtggcagcaggggaacgtcttctcatgctccgtgatgcatgaggctctgcacaaccactacacgcagaagagcctctccctgtctccgggtaaa

SEQ ID NO: 972 - DNA, 336 bp, Artificial
  Humanized antibody sequence
gaggtgcagcttgtggagtctgggggaggcttggtccagcctggggggtccctgagactctcctgtgcagcctctggaatcgacctcaatagctactacatgacctgggtccgtcaggctccagggaaggggctggagtggatcggattcattgatgctggtggtgacgcatactacgcgagctgggcgaaaggccgattcaccatctccagagacaattccaagaacaccgtgtatcttcaaatgaacagcctgagagctgaggacactgctgtgtatttctgtgctagagatcttgacttgtggggccaagggaccctcgtcaccgtctcgagc

SEQ ID NO: 973 - DNA, 90 bp, Artificial
  Humanized antibody sequence
gaggtgcagcttgtggagtctgggggaggcttggtccagcctggggggtccctgagactctcctgtgcagcctctggaatcgacctcaat

SEQ ID NO: 974 - DNA, 15 bp, Oryctolagus cuniculus
agctactacatgacc

SEQ ID NO: 975 - DNA, 42 bp, Artificial
  Humanized antibody sequence
tgggtccgtcaggctccagggaaggggctggagtggatcgga

SEQ ID NO: 976 - DNA, 48 bp, Oryctolagus cuniculus; identical to SEQ ID NO: 416

SEQ ID NO: 977 - DNA, 96 bp, Artificial
  Humanized antibody sequence
cgattcaccatctccagagacaattccaagaacaccgtgtatcttcaaatgaacagcctgagagctgaggacactgctgtgtatttctgtgctaga

SEQ ID NO: 978 - DNA, 12 bp, Oryctolagus cuniculus
gatcttgacttg

SEQ ID NO: 979 - DNA, 33 bp, Artificial
  Humanized antibody sequence
tggggccaagggaccctcgtcaccgtctcgagc

SEQ ID NO: 980 - DNA, 990 bp, Artificial; identical to SEQ ID NO: 460
  Humanized antibody sequence

SEQ ID NO: 981 - protein, 216 aa, Artificial
  Humanized antibody sequence
DAQLTQSPSTLSASVGDRVTITCQSSESVYGNYLAWFQQKPGKAPKFLIYEASKLESGVPSRFSGSGSGTEFTLTISSLQPDDFATYYCAGGDISEGVAFGGGTKVEIKRTVAAPSVFIFPPSDEQLKSGTASVVCLLNNFYPREAKVQWKVDNALQSGNSQESVTEQDSKDSTYSLSSTLTLSKADYEKHKVYACEVTHQGLSSPVTKSFNRGEC

SEQ ID NO: 982 - protein, 110 aa, Artificial
  Humanized antibody sequence
DAQLTQSPSTLSASVGDRVTITCQSSESVYGNYLAWFQQKPGKAPKFLIYEASKLESGVPSRFSGSGSGTEFTLTISSLQPDDFATYYCAGGDISEGVAFGGGTKVEIKR

SEQ ID NO: 983 - protein, 23 aa, Artificial
  Humanized antibody sequence
DAQLTQSPSTLSASVGDRVTITC

SEQ ID NO: 984 - protein, 12 aa, Oryctolagus cuniculus
QSSESVYGNYLA

SEQ ID NO: 985 - protein, 15 aa, Artificial
  Humanized antibody sequence
WFQQKPGKAPKFLIY

SEQ ID NO: 986 - protein, 7 aa, Oryctolagus cuniculus
EASKLES

SEQ ID NO: 987 - protein, 32 aa, Artificial
  Humanized antibody sequence
GVPSRFSGSGSGTEFTLTISSLQPDDFATYYC

SEQ ID NO: 988 - protein, 10 aa, Oryctolagus cuniculus
AGGDISEGVA

SEQ ID NO: 989 - protein, 11 aa, Artificial
  Humanized antibody sequence
FGGGTKVEIKR

SEQ ID NO: 990 - protein, 106 aa, Artificial; identical to SEQ ID NO: 430
  Humanized antibody sequence

SEQ ID NO: 991 - DNA, 648 bp, Artificial
  Humanized antibody sequence
gacgcccagctgacccagtctccttccaccctgtctgcatctgtaggagacagagtcaccatcacttgtcagtccagtgagagtgtttacggtaactacttagcctggtttcagcagaaaccaggaaaagcccctaagttcctgatctatgaagcatccaaactggaatctggagtcccatcaaggttcagcggcagtggatctggaacagaattcactctcaccatcagcagcctgcagcctgatgattttgcaacttactactgtgcaggcggtgatattagtgaaggtgttgctttcggcggaggaaccaaggtggaaatcaaacgtacggtagcggccccatctgtcttcatcttcccgccatctgatgagcagttgaaatctggaactgcctctgttgtgtgcctgctgaataacttctatcccagagaggccaaagtacagtggaaggtggataacgccctccaatcgggtaactcccaggagagtgtcacagagcaggacagcaaggacagcacctacagcctcagcagcaccctgacgctgagcaaagcagactacgagaaacacaaagtctacgcctgcgaagtcacccatcagggcctgagctcgcccgtcacaaagagcttcaacaggggagagtgt

SEQ ID NO: 992 - DNA, 330 bp, Artificial
  Humanized antibody sequence
gacgcccagctgacccagtctccttccaccctgtctgcatctgtaggagacagagtcaccatcacttgtcagtccagtgagagtgtttacggtaactacttagcctggtttcagcagaaaccaggaaaagcccctaagttcctgatctatgaagcatccaaactggaatctggagtcccatcaaggttcagcggcagtggatctggaacagaattcactctcaccatcagcagcctgcagcctgatgattttgcaacttactactgtgcaggcggtgatattagtgaaggtgttgctttcggcggaggaaccaaggtggaaatcaaacgt

SEQ ID NO: 993 - DNA, 69 bp, Artificial
  Humanized antibody sequence
gacgcccagctgacccagtctccttccaccctgtctgcatctgtaggagacagagtcaccatcacttgt

SEQ ID NO: 994 - DNA, 36 bp, Oryctolagus cuniculus; identical to SEQ ID NO: 434

SEQ ID NO: 995 - DNA, 45 bp, Artificial
  Humanized antibody sequence
tggtttcagcagaaaccaggaaaagcccctaagttcctgatctat

SEQ ID NO: 996 - DNA, 21 bp, Oryctolagus cuniculus
gaagcatccaaactggaatct

SEQ ID NO: 997 - DNA, 96 bp, Artificial
  Humanized antibody sequence
ggagtcccatcaaggttcagcggcagtggatctggaacagaattcactctcaccatcagcagcctgcagcctgatgattttgcaacttactactgt

SEQ ID NO: 998 - DNA, 30 bp, Oryctolagus cuniculus; identical to SEQ ID NO: 438

SEQ ID NO: 999 - DNA, 33 bp, Artificial
  Humanized antibody sequence
ttcggcggaggaaccaaggtggaaatcaaacgt

SEQ ID NO: 1000 - DNA, 318 bp, Artificial; identical to SEQ ID NO: 440
  Humanized antibody sequence

SEQ ID NO: 1001-1200 - skipped (200 entries)

SEQ ID NO: 1201 - protein, 442 aa, Artificial
  Humanized antibody sequence
EVQLVESGGGLVQPGGSLRLSCAASGIDLSSYYMTWVRQAPGKGLEWIGFIDAGGSAYYATWAKGRFTISRDNSKNTVYLQMNSLRAEDTAVYFCARDLDLWGQGTLVTVSSASTKGPSVFPLAPSSKSTSGGTAALGCLVKDYFPEPVTVSWNSGALTSGVHTFPAVLQSSGLYSLSSVVTVPSSSLGTQTYICNVNHKPSNTKVDKKVEPKSCDKTHTCPPCPAPELLGGPSVFLFPPKPKDTLMISRTPEVTCVVVDVSHEDPEVKFNWYVDGVEVHNAKTKPREEQYASTYRVVSVLTVLHQDWLNGKEYKCKVSNKALPAPIEKTISKAKGQPREPQVYTLPPSREEMTKNQVSLTCLVKGFYPSDIAVEWESNGQPENNYKTTPPVLDSDGSFFLYSKLTVDKSRWQQGNVFSCSVMHEALHNHYTQKSLSLSPGK

SEQ ID NO: 1202 - protein, 112 aa, Artificial
  Humanized antibody sequence
EVQLVESGGGLVQPGGSLRLSCAASGIDLSSYYMTWVRQAPGKGLEWIGFIDAGGSAYYATWAKGRFTISRDNSKNTVYLQMNSLRAEDTAVYFCARDLDLWGQGTLVTVSS

SEQ ID NO: 1203 - protein, 30 aa, Artificial
  Humanized antibody sequence
EVQLVESGGGLVQPGGSLRLSCAASGIDLS

SEQ ID NO: 1204 - protein, 5 aa, Oryctolagus cuniculus
SYYMT

SEQ ID NO: 1205 - protein, 14 aa, Artificial
  Humanized antibody sequence
WVRQAPGKGLEWIG

SEQ ID NO: 1206 - protein, 16 aa, Oryctolagus cuniculus
FIDAGGSAYYATWAKG

SEQ ID NO: 1207 - protein, 32 aa, Artificial; identical to SEQ ID NO: 967
  Humanized antibody sequence

SEQ ID NO: 1208 - protein, 4 aa, Oryctolagus cuniculus
DLDL

SEQ ID NO: 1209 - protein, 11 aa, Artificial
  Humanized antibody sequence
WGQGTLVTVSS

SEQ ID NO: 1210 - protein, 330 aa, Artificial; identical to SEQ ID NO: 450
  Humanized antibody sequence

SEQ ID NO: 1211 - DNA, 1326 bp, Artificial
  Humanized antibody sequence
gaggtgcagcttgtggagtctgggggaggcttggtccagcctggggggtccctgagactctcctgtgcagcctctggaatcgacctcagtagctactacatgacctgggtccgtcaggctccagggaaggggctggagtggatcggattcattgatgctggtggtagcgcatactacgcgacctgggcaaaaggccgattcaccatctccagagacaattccaagaacaccgtgtatcttcaaatgaacagcctgagagctgaggacactgctgtgtatttctgtgctagagatcttgacttgtggggccaagggaccctcgtcaccgtctcgagcgcctccaccaagggcccatcggtcttccccctggcaccctcctccaagagcacctctgggggcacagcggccctgggctgcctggtcaaggactacttccccgaaccggtgacggtgtcgtggaactcaggcgccctgaccagcggcgtgcacaccttcccggctgtcctacagtcctcaggactctactccctcagcagcgtggtgaccgtgccctccagcagcttgggcacccagacctacatctgcaacgtgaatcacaagcccagcaacaccaaggtggacaagaaagttgagcccaaatcttgtgacaaaactcacacatgcccaccgtgcccagcacctgaactcctggggggaccgtcagtcttcctcttccccccaaaacccaaggacaccctcatgatctcccggacccctgaggtcacatgcgtggtggtggacgtgagccacgaagaccctgaggtcaagttcaactggtacgtggacggcgtggaggtgcataatgccaagacaaagccgcgggaggagcagtacgccagcacgtaccgtgtggtcagcgtcctcaccgtcctgcaccaggactggctgaatggcaaggagtacaagtgcaaggtctccaacaaagccctcccagcccccatcgagaaaaccatctccaaagccaaagggcagccccgagaaccacaggtgtacaccctgcccccatcccgggaggagatgaccaagaaccaggtcagcctgacctgcctggtcaaaggcttctatcccagcgacatcgccgtggagtgggagagcaatgggcagccggagaacaactacaagaccacgcctcccgtgctggactccgacggctccttcttcctctacagcaagctcaccgtggacaagagcaggtggcagcaggggaacgtcttctcatgctccgtgatgcatgaggctctgcacaaccactacacgcagaagagcctctccctgtctccgggtaaa

SEQ ID NO: 1212 - DNA, 336 bp, Artificial
  Humanized antibody sequence
gaggtgcagcttgtggagtctgggggaggcttggtccagcctggggggtccctgagactctcctgtgcagcctctggaatcgacctcagtagctactacatgacctgggtccgtcaggctccagggaaggggctggagtggatcggattcattgatgctggtggtagcgcatactacgcgacctgggcaaaaggccgattcaccatctccagagacaattccaagaacaccgtgtatcttcaaatgaacagcctgagagctgaggacactgctgtgtatttctgtgctagagatcttgacttgtggggccaagggaccctcgtcaccgtctcgagc

SEQ ID NO: 1213 - DNA, 90 bp, Artificial
  Humanized antibody sequence
gaggtgcagcttgtggagtctgggggaggcttggtccagcctggggggtccctgagactctcctgtgcagcctctggaatcgacctcagt

SEQ ID NO: 1214 - DNA, 15 bp, Oryctolagus cuniculus
agctactacatgacc

SEQ ID NO: 1215 - DNA, 42 bp, Artificial; identical to SEQ ID NO: 975
  Humanized antibody sequence

SEQ ID NO: 1216 - DNA, 48 bp, Oryctolagus cuniculus; identical to SEQ ID NO: 856

SEQ ID NO: 1217 - DNA, 96 bp, Artificial; identical to SEQ ID NO: 977
  Humanized antibody sequence

SEQ ID NO: 1218 - DNA, 12 bp, Oryctolagus cuniculus
gatcttgacttg

SEQ ID NO: 1219 - DNA, 33 bp, Artificial; identical to SEQ ID NO: 979
  Humanized antibody sequence

SEQ ID NO: 1220 - DNA, 990 bp, Artificial; identical to SEQ ID NO: 460
  Humanized antibody sequence

SEQ ID NO: 1221 - protein, 216 aa, Artificial
  Humanized antibody sequence
DAQLTQSPSTLSASVGDRVTITCKSSESVYGDYLAWFQQKPGKAPKQLIYDASTLASGVPSRFSGSGSGTEFTLTISSLQPDDFATYYCAGGYVSAGVAFGGGTKVEIKRTVAAPSVFIFPPSDEQLKSGTASVVCLLNNFYPREAKVQWKVDNALQSGNSQESVTEQDSKDSTYSLSSTLTLSKADYEKHKVYACEVTHQGLSSPVTKSFNRGEC

SEQ ID NO: 1222 - protein, 110 aa, Artificial
  Humanized antibody sequence
DAQLTQSPSTLSASVGDRVTITCKSSESVYGDYLAWFQQKPGKAPKQLIYDASTLASGVPSRFSGSGSGTEFTLTISSLQPDDFATYYCAGGYVSAGVAFGGGTKVEIKR

SEQ ID NO: 1223 - protein, 23 aa, Artificial
  Humanized antibody sequence
DAQLTQSPSTLSASVGDRVTITC

SEQ ID NO: 1224 - protein, 12 aa, Oryctolagus cuniculus
KSSESVYGDYLA

SEQ ID NO: 1225 - protein, 15 aa, Artificial
  Humanized antibody sequence
WFQQKPGKAPKQLIY

SEQ ID NO: 1226 - protein, 7 aa, Oryctolagus cuniculus
DASTLAS

SEQ ID NO: 1227 - protein, 32 aa, Artificial; identical to SEQ ID NO: 987
  Humanized antibody sequence

SEQ ID NO: 1228 - protein, 10 aa, Oryctolagus cuniculus
AGGYVSAGVA

SEQ ID NO: 1229 - protein, 11 aa, Artificial
  Humanized antibody sequence
FGGGTKVEIKR

SEQ ID NO: 1230 - protein, 106 aa, Artificial; identical to SEQ ID NO: 430
  Humanized antibody sequence

SEQ ID NO: 1231 - DNA, 648 bp, Artificial
  Humanized antibody sequence
gacgcccagctgacccagtctccttccaccctgtctgcatctgtaggagacagagtcaccatcacttgtaagtccagtgagagcgtttatggtgactacttagcctggtttcagcagaaaccaggaaaagcccctaagcaactgatctatgatgcatccactctggcatctggagtcccatcaaggttcagcggcagtggatctggaacagaattcactctcaccatcagcagcctgcagcctgatgattttgcaacttactactgtgcaggcggttatgttagtgcaggtgttgctttcggcggaggaaccaaggtggaaatcaaacgtacggtagcggccccatctgtcttcatcttcccgccatctgatgagcagttgaaatctggaactgcctctgttgtgtgcctgctgaataacttctatcccagagaggccaaagtacagtggaaggtggataacgccctccaatcgggtaactcccaggagagtgtcacagagcaggacagcaaggacagcacctacagcctcagcagcaccctgacgctgagcaaagcagactacgagaaacacaaagtctacgcctgcgaagtcacccatcagggcctgagctcgcccgtcacaaagagcttcaacaggggagagtgt

SEQ ID NO: 1232 - DNA, 330 bp, Artificial
  Humanized antibody sequence
gacgcccagctgacccagtctccttccaccctgtctgcatctgtaggagacagagtcaccatcacttgtaagtccagtgagagcgtttatggtgactacttagcctggtttcagcagaaaccaggaaaagcccctaagcaactgatctatgatgcatccactctggcatctggagtcccatcaaggttcagcggcagtggatctggaacagaattcactctcaccatcagcagcctgcagcctgatgattttgcaacttactactgtgcaggcggttatgttagtgcaggtgttgctttcggcggaggaaccaaggtggaaatcaaacgt

SEQ ID NO: 1233 - DNA, 69 bp, Artificial; identical to SEQ ID NO: 993
  Humanized antibody sequence

SEQ ID NO: 1234 - DNA, 36 bp, Oryctolagus cuniculus; identical to SEQ ID NO: 874

SEQ ID NO: 1235 - DNA, 45 bp, Artificial
  Humanized antibody sequence
tggtttcagcagaaaccaggaaaagcccctaagcaactgatctat

SEQ ID NO: 1236 - DNA, 21 bp, Oryctolagus cuniculus
gatgcatccactctggcatct

SEQ ID NO: 1237 - DNA, 96 bp, Artificial; identical to SEQ ID NO: 997
  Humanized antibody sequence

SEQ ID NO: 1238 - DNA, 30 bp, Oryctolagus cuniculus; identical to SEQ ID NO: 878

SEQ ID NO: 1239 - DNA, 33 bp, Artificial; identical to SEQ ID NO: 999
  Humanized antibody sequence

SEQ ID NO: 1240 - DNA, 318 bp, Artificial; identical to SEQ ID NO: 440
  Humanized antibody sequence

SEQ ID NO: 1241 - protein, 38 aa, Homo sapiens
  MOD_RES (38)..(38): AMIDATION
HSDGIFTDSYSRYRKQMAVKKYLAAVLGKRYKQRVKNK

SEQ ID NO: 1242 - protein, 27 aa, Homo sapiens
  MOD_RES (27)..(27): AMIDATION
HSDGIFTDSYSRYRKQMAVKKYLAAVL

SEQ ID NO: 1243 - protein, 28 aa, Homo sapiens
  MOD_RES (28)..(28): AMIDATION
HSDAVFTDNYTRLRKQMAVKKYLNSILN

SEQ ID NO: 1244 - protein, 330 aa, Artificial
  Humanized antibody sequence
ASTKGPSVFPLAPSSKSTSGGTAALGCLVKDYFPEPVTVSWNSGALTSGVHTFPAVLQSSGLYSLSSVVTVPSSSLGTQTYICNVNHKPSNTKVDKRVEPKSCDKTHTCPPCPAPELLGGPSVFLFPPKPKDTLMISRTPEVTCVVVDVSHEDPEVKFNWYVDGVEVHNAKTKPREEQYASTYRVVSVLTVLHQDWLNGKEYKCKVSNKALPAPIEKTISKAKGQPREPQVYTLPPSREEMTKNQVSLTCLVKGFYPSDIAVEWESNGQPENNYKTTPPVLDSDGSFFLYSKLTVDKSRWQQGNVFSCSVMHEALHNHYTQKSLSLSPGK

SEQ ID NO: 1245 - protein, 330 aa, Artificial; identical to SEQ ID NO: 410
  Humanized antibody sequence

SEQ ID NO: 1246 - protein, 330 aa, Artificial; identical to SEQ ID NO: 450
  Humanized antibody sequence

SEQ ID NO: 1247-1280 - skipped (34 entries)

SEQ ID NO: 1281 - protein, 442 aa, Artificial; identical to SEQ ID NO: 961
  Humanized Antibody

SEQ ID NO: 1282 - protein, 112 aa, Artificial; identical to SEQ ID NO: 962
  Humanized Antibody

SEQ ID NO: 1283 - protein, 30 aa, Artificial; identical to SEQ ID NO: 963
  Humanized Antibody

SEQ ID NO: 1284 - protein, 5 aa, Oryctolagus cuniculus
SYYMT

SEQ ID NO: 1285 - protein, 14 aa, Artificial
  Humanized Antibody
WVRQAPGKGLEWIG

SEQ ID NO: 1286 - protein, 16 aa, Oryctolagus cuniculus
FIDAGGDAYYASWAKG

SEQ ID NO: 1287 - protein, 32 aa, Artificial; identical to SEQ ID NO: 967
  Humanized Antibody

SEQ ID NO: 1288 - protein, 4 aa, Oryctolagus cuniculus
DLDL

SEQ ID NO: 1289 - protein, 11 aa, Artificial
  Humanized Antibody
WGQGTLVTVSS

SEQ ID NO: 1290 - protein, 330 aa, Artificial; identical to SEQ ID NO: 450
  Humanized Antibody

SEQ ID NO: 1291 - DNA, 1326 bp, Artificial; identical to SEQ ID NO: 971
  Humanized Antibody

SEQ ID NO: 1292 - DNA, 336 bp, Artificial; identical to SEQ ID NO: 972
  Humanized Antibody

SEQ ID NO: 1293 - DNA, 90 bp, Artificial; identical to SEQ ID NO: 973
  Humanized Antibody

SEQ ID NO: 1294 - DNA, 15 bp, Oryctolagus cuniculus
agctactacatgacc

SEQ ID NO: 1295 - DNA, 42 bp, Artificial; identical to SEQ ID NO: 975
  Humanized Antibody

SEQ ID NO: 1296 - DNA, 48 bp, Oryctolagus cuniculus; identical to SEQ ID NO: 416

SEQ ID NO: 1297 - DNA, 96 bp, Artificial; identical to SEQ ID NO: 977
  Humanized Antibody

SEQ ID NO: 1298 - DNA, 12 bp, Oryctolagus cuniculus
gatcttgacttg

SEQ ID NO: 1299 - DNA, 33 bp, Artificial; identical to SEQ ID NO: 979
  Humanized Antibody

SEQ ID NO: 1300 - DNA, 990 bp, Artificial; identical to SEQ ID NO: 460
  Humanized Antibody

SEQ ID NO: 1301 - protein, 215 aa, Artificial
  Humanized Antibody
AVLTQSPSTLSASVGDRVTITCQSSESVYGNYLAWFQQKPGKAPKFLIYEASKLESGVPSRFSGSGSGTEFTLTISSLQPDDFATYYCAGGDISEGVAFGGGTKVEIKRTVAAPSVFIFPPSDEQLKSGTASVVCLLNNFYPREAKVQWKVDNALQSGNSQESVTEQDSKDSTYSLSSTLTLSKADYEKHKVYACEVTHQGLSSPVTKSFNRGEC

SEQ ID NO: 1302 - protein, 109 aa, Artificial
  Humanized Antibody
AVLTQSPSTLSASVGDRVTITCQSSESVYGNYLAWFQQKPGKAPKFLIYEASKLESGVPSRFSGSGSGTEFTLTISSLQPDDFATYYCAGGDISEGVAFGGGTKVEIKR

SEQ ID NO: 1303 - protein, 22 aa, Artificial
  Humanized Antibody
AVLTQSPSTLSASVGDRVTITC

SEQ ID NO: 1304 - protein, 12 aa, Oryctolagus cuniculus
QSSESVYGNYLA

SEQ ID NO: 1305 - protein, 15 aa, Artificial
  Humanized Antibody
WFQQKPGKAPKFLIY

SEQ ID NO: 1306 - protein, 7 aa, Oryctolagus cuniculus
EASKLES

SEQ ID NO: 1307 - protein, 32 aa, Artificial; identical to SEQ ID NO: 987
  Humanized Antibody

SEQ ID NO: 1308 - protein, 10 aa, Oryctolagus cuniculus
AGGDISEGVA

SEQ ID NO: 1309 - protein, 11 aa, Artificial
  Humanized Antibody
FGGGTKVEIKR

SEQ ID NO: 1310 - protein, 106 aa, Artificial; identical to SEQ ID NO: 430
  Humanized Antibody

SEQ ID NO: 1311 - DNA, 645 bp, Artificial
  Humanized Antibody
gccgtgctgacccagtctccttccaccctgtctgcatctgtaggagacagagtcaccatcacttgtcagtccagtgagagtgtttacggtaactacttagcctggtttcagcagaaaccaggaaaagcccctaagttcctgatctatgaagcatccaaactggaatctggagtcccatcaaggttcagcggcagtggatctggaacagaattcactctcaccatcagcagcctgcagcctgatgattttgcaacttactactgtgcaggcggtgatattagtgaaggtgttgctttcggcggaggaaccaaggtggaaatcaaacgtacggtagcggccccatctgtcttcatcttcccgccatctgatgagcagttgaaatctggaactgcctctgttgtgtgcctgctgaataacttctatcccagagaggccaaagtacagtggaaggtggataacgccctccaatcgggtaactcccaggagagtgtcacagagcaggacagcaaggacagcacctacagcctcagcagcaccctgacgctgagcaaagcagactacgagaaacacaaagtctacgcctgcgaagtcacccatcagggcctgagctcgcccgtcacaaagagcttcaacaggggagagtgt

SEQ ID NO: 1312 - DNA, 327 bp, Artificial
  Humanized Antibody
gccgtgctgacccagtctccttccaccctgtctgcatctgtaggagacagagtcaccatcacttgtcagtccagtgagagtgtttacggtaactacttagcctggtttcagcagaaaccaggaaaagcccctaagttcctgatctatgaagcatccaaactggaatctggagtcccatcaaggttcagcggcagtggatctggaacagaattcactctcaccatcagcagcctgcagcctgatgattttgcaacttactactgtgcaggcggtgatattagtgaaggtgttgctttcggcggaggaaccaaggtggaaatcaaacgt

SEQ ID NO: 1313 - DNA, 66 bp, Artificial
  Humanized Antibody
gccgtgctgacccagtctccttccaccctgtctgcatctgtaggagacagagtcaccatcacttgt

SEQ ID NO: 1314 - DNA, 36 bp, Oryctolagus cuniculus; identical to SEQ ID NO: 434

SEQ ID NO: 1315 - DNA, 45 bp, Artificial; identical to SEQ ID NO: 995
  Humanized Antibody

SEQ ID NO: 1316 - DNA, 21 bp, Oryctolagus cuniculus
gaagcatccaaactggaatct

SEQ ID NO: 1317 - DNA, 96 bp, Artificial; identical to SEQ ID NO: 997
  Humanized Antibody

SEQ ID NO: 1318 - DNA, 30 bp, Oryctolagus cuniculus; identical to SEQ ID NO: 438

SEQ ID NO: 1319 - DNA, 33 bp, Artificial; identical to SEQ ID NO: 999
  Humanized Antibody

SEQ ID NO: 1320 - DNA, 318 bp, Artificial; identical to SEQ ID NO: 440
  Humanized Antibody

SEQ ID NO: 1321 - protein, 442 aa, Artificial; identical to SEQ ID NO: 961
  Humanized Antibody

SEQ ID NO: 1322 - protein, 112 aa, Artificial; identical to SEQ ID NO: 962
  Humanized Antibody

SEQ ID NO: 1323 - protein, 30 aa, Artificial; identical to SEQ ID NO: 963
  Humanized Antibody

SEQ ID NO: 1324 - protein, 5 aa, Oryctolagus cuniculus
SYYMT

SEQ ID NO: 1325 - protein, 14 aa, Artificial
  Humanized Antibody
WVRQAPGKGLEWIG

SEQ ID NO: 1326 - protein, 16 aa, Oryctolagus cuniculus
FIDAGGDAYYASWAKG

SEQ ID NO: 1327 - protein, 32 aa, Artificial; identical to SEQ ID NO: 967
  Humanized Antibody

SEQ ID NO: 1328 - protein, 4 aa, Oryctolagus cuniculus
DLDL

SEQ ID NO: 1329 - protein, 11 aa, Artificial
  Humanized Antibody
WGQGTLVTVSS

SEQ ID NO: 1330 - protein, 330 aa, Artificial; identical to SEQ ID NO: 450
  Humanized Antibody

SEQ ID NO: 1331 - DNA, 1326 bp, Artificial; identical to SEQ ID NO: 971
  Humanized Antibody

SEQ ID NO: 1332 - DNA, 336 bp, Artificial; identical to SEQ ID NO: 972
  Humanized Antibody

SEQ ID NO: 1333 - DNA, 90 bp, Artificial; identical to SEQ ID NO: 973
  Humanized Antibody

SEQ ID NO: 1334 - DNA, 15 bp, Oryctolagus cuniculus
agctactacatgacc

SEQ ID NO: 1335 - DNA, 42 bp, Artificial; identical to SEQ ID NO: 975
  Humanized Antibody

SEQ ID NO: 1336 - DNA, 48 bp, Oryctolagus cuniculus; identical to SEQ ID NO: 416

SEQ ID NO: 1337 - DNA, 96 bp, Artificial; identical to SEQ ID NO: 977
  Humanized Antibody

SEQ ID NO: 1338 - DNA, 12 bp, Oryctolagus cuniculus
gatcttgacttg

SEQ ID NO: 1339 - DNA, 33 bp, Artificial; identical to SEQ ID NO: 979
  Humanized Antibody

SEQ ID NO: 1340 - DNA, 990 bp, Artificial; identical to SEQ ID NO: 460
  Humanized Antibody

SEQ ID NO: 1341 - protein, 216 aa, Artificial
  Humanized Antibody
DIQLTQSPSTLSASVGDRVTITCQSSESVYGNYLAWFQQKPGKAPKFLIYEASKLESGVPSRFSGSGSGTEFTLTISSLQPDDFATYYCAGGDISEGVAFGGGTKVEIKRTVAAPSVFIFPPSDEQLKSGTASVVCLLNNFYPREAKVQWKVDNALQSGNSQESVTEQDSKDSTYSLSSTLTLSKADYEKHKVYACEVTHQGLSSPVTKSFNRGEC

SEQ ID NO: 1342 - protein, 110 aa, Artificial
  Humanized Antibody
DIQLTQSPSTLSASVGDRVTITCQSSESVYGNYLAWFQQKPGKAPKFLIYEASKLESGVPSRFSGSGSGTEFTLTISSLQPDDFATYYCAGGDISEGVAFGGGTKVEIKR

SEQ ID NO: 1343 - protein, 23 aa, Artificial
  Humanized Antibody
DIQLTQSPSTLSASVGDRVTITC

SEQ ID NO: 1344 - protein, 12 aa, Oryctolagus cuniculus
QSSESVYGNYLA

SEQ ID NO: 1345 - protein, 15 aa, Artificial
  Humanized Antibody
WFQQKPGKAPKFLIY

SEQ ID NO: 1346 - protein, 7 aa, Oryctolagus cuniculus
EASKLES

SEQ ID NO: 1347 - protein, 32 aa, Artificial; identical to SEQ ID NO: 987
  Humanized Antibody

SEQ ID NO: 1348 - protein, 10 aa, Oryctolagus cuniculus
AGGDISEGVA

SEQ ID NO: 1349 - protein, 11 aa, Artificial
  Humanized Antibody
FGGGTKVEIKR

SEQ ID NO: 1350 - protein, 106 aa, Artificial; identical to SEQ ID NO: 430
  Humanized Antibody

SEQ ID NO: 1351 - DNA, 648 bp, Artificial
  Humanized Antibody
gacatccagctgacccagtctccttccaccctgtctgcatctgtaggagacagagtcaccatcacttgtcagtccagtgagagtgtttacggtaactacttagcctggtttcagcagaaaccaggaaaagcccctaagttcctgatctatgaagcatccaaactggaatctggagtcccatcaaggttcagcggcagtggatctggaacagaattcactctcaccatcagcagcctgcagcctgatgattttgcaacttactactgtgcaggcggtgatattagtgaaggtgttgctttcggcggaggaaccaaggtggaaatcaaacgtacggtagcggccccatctgtcttcatcttcccgccatctgatgagcagttgaaatctggaactgcctctgttgtgtgcctgctgaataacttctatcccagagaggccaaagtacagtggaaggtggataacgccctccaatcgggtaactcccaggagagtgtcacagagcaggacagcaaggacagcacctacagcctcagcagcaccctgacgctgagcaaagcagactacgagaaacacaaagtctacgcctgcgaagtcacccatcagggcctgagctcgcccgtcacaaagagcttcaacaggggagagtgt

SEQ ID NO: 1352 - DNA, 330 bp, Artificial
  Humanized Antibody
gacatccagctgacccagtctccttccaccctgtctgcatctgtaggagacagagtcaccatcacttgtcagtccagtgagagtgtttacggtaactacttagcctggtttcagcagaaaccaggaaaagcccctaagttcctgatctatgaagcatccaaactggaatctggagtcccatcaaggttcagcggcagtggatctggaacagaattcactctcaccatcagcagcctgcagcctgatgattttgcaacttactactgtgcaggcggtgatattagtgaaggtgttgctttcggcggaggaaccaaggtggaaatcaaacgt

SEQ ID NO: 1353 - DNA, 69 bp, Artificial
  Humanized Antibody
gacatccagctgacccagtctccttccaccctgtctgcatctgtaggagacagagtcaccatcacttgt

SEQ ID NO: 1354 - DNA, 36 bp, Oryctolagus cuniculus; identical to SEQ ID NO: 434

SEQ ID NO: 1355 - DNA, 45 bp, Artificial; identical to SEQ ID NO: 995
  Humanized Antibody

SEQ ID NO: 1356 - DNA, 21 bp, Oryctolagus cuniculus
gaagcatccaaactggaatct

SEQ ID NO: 1357 - DNA, 96 bp, Artificial; identical to SEQ ID NO: 997
  Humanized Antibody

SEQ ID NO: 1358 - DNA, 30 bp, Oryctolagus cuniculus; identical to SEQ ID NO: 438

SEQ ID NO: 1359 - DNA, 33 bp, Artificial; identical to SEQ ID NO: 999
  Humanized Antibody

SEQ ID NO: 1360 - DNA, 318 bp, Artificial; identical to SEQ ID NO: 440
  Humanized Antibody

SEQ ID NO: 1361 - protein, 442 aa, Artificial; identical to SEQ ID NO: 961
  Humanized Antibody

SEQ ID NO: 1362 - protein, 112 aa, Artificial; identical to SEQ ID NO: 962
  Humanized Antibody

SEQ ID NO: 1363 - protein, 30 aa, Artificial; identical to SEQ ID NO: 963
  Humanized Antibody

SEQ ID NO: 1364 - protein, 5 aa, Oryctolagus cuniculus
SYYMT

SEQ ID NO: 1365 - protein, 14 aa, Artificial
  Humanized Antibody
WVRQAPGKGLEWIG

SEQ ID NO: 1366 - protein, 16 aa, Oryctolagus cuniculus
FIDAGGDAYYASWAKG

SEQ ID NO: 1367 - protein, 32 aa, Artificial; identical to SEQ ID NO: 967
  Humanized Antibody

SEQ ID NO: 1368 - protein, 4 aa, Oryctolagus cuniculus
DLDL

SEQ ID NO: 1369 - protein, 11 aa, Artificial
  Humanized Antibody
WGQGTLVTVSS

SEQ ID NO: 1370 - protein, 330 aa, Artificial; identical to SEQ ID NO: 450
  Humanized Antibody

SEQ ID NO: 1371 - DNA, 1326 bp, Artificial; identical to SEQ ID NO: 971
  Humanized Antibody

SEQ ID NO: 1372 - DNA, 336 bp, Artificial; identical to SEQ ID NO: 972
  Humanized Antibody

SEQ ID NO: 1373 - DNA, 90 bp, Artificial; identical to SEQ ID NO: 973
  Humanized Antibody

SEQ ID NO: 1374 - DNA, 15 bp, Oryctolagus cuniculus
agctactacatgacc

SEQ ID NO: 1375 - DNA, 42 bp, Artificial; identical to SEQ ID NO: 975
  Humanized Antibody

SEQ ID NO: 1376 - DNA, 48 bp, Oryctolagus cuniculus; identical to SEQ ID NO: 416

SEQ ID NO: 1377 - DNA, 96 bp, Artificial; identical to SEQ ID NO: 977
  Humanized Antibody

SEQ ID NO: 1378 - DNA, 12 bp, Oryctolagus cuniculus
gatcttgacttg

SEQ ID NO: 1379 - DNA, 33 bp, Artificial; identical to SEQ ID NO: 979
  Humanized Antibody

SEQ ID NO: 1380 - DNA, 990 bp, Artificial; identical to SEQ ID NO: 460
  Humanized Antibody

SEQ ID NO: 1381 - protein, 216 aa, Artificial
  Humanized Antibody
DIVLTQSPSTLSASVGDRVTITCQSSESVYGNYLAWFQQKPGKAPKFLIYEASKLESGVPSRFSGSGSGTEFTLTISSLQPDDFATYYCAGGDISEGVAFGGGTKVEIKRTVAAPSVFIFPPSDEQLKSGTASVVCLLNNFYPREAKVQWKVDNALQSGNSQESVTEQDSKDSTYSLSSTLTLSKADYEKHKVYACEVTHQGLSSPVTKSFNRGEC

SEQ ID NO: 1382 - protein, 110 aa, Artificial
  Humanized Antibody
DIVLTQSPSTLSASVGDRVTITCQSSESVYGNYLAWFQQKPGKAPKFLIYEASKLESGVPSRFSGSGSGTEFTLTISSLQPDDFATYYCAGGDISEGVAFGGGTKVEIKR

SEQ ID NO: 1383 - protein, 23 aa, Artificial
  Humanized Antibody
DIVLTQSPSTLSASVGDRVTITC

SEQ ID NO: 1384 - protein, 12 aa, Oryctolagus cuniculus
QSSESVYGNYLA

SEQ ID NO: 1385 - protein, 15 aa, Artificial
  Humanized Antibody
WFQQKPGKAPKFLIY

SEQ ID NO: 1386 - protein, 7 aa, Oryctolagus cuniculus
EASKLES

SEQ ID NO: 1387 - protein, 32 aa, Artificial; identical to SEQ ID NO: 987
  Humanized Antibody

SEQ ID NO: 1388 - protein, 10 aa, Oryctolagus cuniculus
AGGDISEGVA

SEQ ID NO: 1389 - protein, 11 aa, Artificial
  Humanized Antibody
FGGGTKVEIKR

SEQ ID NO: 1390 - protein, 106 aa, Artificial; identical to SEQ ID NO: 430
  Humanized Antibody

SEQ ID NO: 1391 - DNA, 648 bp, Artificial
  Humanized Antibody
gacatcgtgctgacccagtctccttccaccctgtctgcatctgtaggagacagagtcaccatcacttgtcagtccagtgagagtgtttacggtaactacttagcctggtttcagcagaaaccaggaaaagcccctaagttcctgatctatgaagcatccaaactggaatctggagtcccatcaaggttcagcggcagtggatctggaacagaattcactctcaccatcagcagcctgcagcctgatgattttgcaacttactactgtgcaggcggtgatattagtgaaggtgttgctttcggcggaggaaccaaggtggaaatcaaacgtacggtagcggccccatctgtcttcatcttcccgccatctgatgagcagttgaaatctggaactgcctctgttgtgtgcctgctgaataacttctatcccagagaggccaaagtacagtggaaggtggataacgccctccaatcgggtaactcccaggagagtgtcacagagcaggacagcaaggacagcacctacagcctcagcagcaccctgacgctgagcaaagcagactacgagaaacacaaagtctacgcctgcgaagtcacccatcagggcctgagctcgcccgtcacaaagagcttcaacaggggagagtgt

SEQ ID NO: 1392 - DNA, 330 bp, Artificial
  Humanized Antibody
gacatcgtgctgacccagtctccttccaccctgtctgcatctgtaggagacagagtcaccatcacttgtcagtccagtgagagtgtttacggtaactacttagcctggtttcagcagaaaccaggaaaagcccctaagttcctgatctatgaagcatccaaactggaatctggagtcccatcaaggttcagcggcagtggatctggaacagaattcactctcaccatcagcagcctgcagcctgatgattttgcaacttactactgtgcaggcggtgatattagtgaaggtgttgctttcggcggaggaaccaaggtggaaatcaaacgt

SEQ ID NO: 1393 - DNA, 69 bp, Artificial
  Humanized Antibody
gacatcgtgctgacccagtctccttccaccctgtctgcatctgtaggagacagagtcaccatcacttgt

SEQ ID NO: 1394 - DNA, 36 bp, Oryctolagus cuniculus; identical to SEQ ID NO: 434

SEQ ID NO: 1395 - DNA, 45 bp, Artificial; identical to SEQ ID NO: 995
  Humanized Antibody

SEQ ID NO: 1396 - DNA, 21 bp, Oryctolagus cuniculus
gaagcatccaaactggaatct

SEQ ID NO: 1397 - DNA, 96 bp, Artificial; identical to SEQ ID NO: 997
  Humanized Antibody

SEQ ID NO: 1398 - DNA, 30 bp, Oryctolagus cuniculus; identical to SEQ ID NO: 438

SEQ ID NO: 1399 - DNA, 33 bp, Artificial; identical to SEQ ID NO: 999
  Humanized Antibody

SEQ ID NO: 1400 - DNA, 318 bp, Artificial; identical to SEQ ID NO: 440
  Humanized Antibody

SEQ ID NO: 1401 - protein, 442 aa, Artificial; identical to SEQ ID NO: 961
  Humanized Antibody

SEQ ID NO: 1402 - protein, 112 aa, Artificial; identical to SEQ ID NO: 962
  Humanized Antibody

SEQ ID NO: 1403 - protein, 30 aa, Artificial; identical to SEQ ID NO: 963
  Humanized Antibody

SEQ ID NO: 1404 - protein, 5 aa, Oryctolagus cuniculus
SYYMT

SEQ ID NO: 1405 - protein, 14 aa, Artificial
  Humanized Antibody
WVRQAPGKGLEWIG

SEQ ID NO: 1406 - protein, 16 aa, Oryctolagus cuniculus
FIDAGGDAYYASWAKG

SEQ ID NO: 1407 - protein, 32 aa, Artificial; identical to SEQ ID NO: 967
  Humanized Antibody

SEQ ID NO: 1408 - protein, 4 aa, Oryctolagus cuniculus
DLDL

SEQ ID NO: 1409 - protein, 11 aa, Artificial
  Humanized Antibody
WGQGTLVTVSS

SEQ ID NO: 1410 - protein, 330 aa, Artificial; identical to SEQ ID NO: 450
  Humanized Antibody

SEQ ID NO: 1411 - DNA, 1326 bp, Artificial; identical to SEQ ID NO: 971
  Humanized Antibody

SEQ ID NO: 1412 - DNA, 336 bp, Artificial; identical to SEQ ID NO: 972
  Humanized Antibody

SEQ ID NO: 1413 - DNA, 90 bp, Artificial; identical to SEQ ID NO: 973
  Humanized Antibody

SEQ ID NO: 1414 - DNA, 15 bp, Oryctolagus cuniculus
agctactacatgacc

SEQ ID NO: 1415 - DNA, 42 bp, Artificial; identical to SEQ ID NO: 975
  Humanized Antibody

SEQ ID NO: 1416 - DNA, 48 bp, Oryctolagus cuniculus; identical to SEQ ID NO: 416

SEQ ID NO: 1417 - DNA, 96 bp, Artificial; identical to SEQ ID NO: 977
  Humanized Antibody

SEQ ID NO: 1418 - DNA, 12 bp, Oryctolagus cuniculus
gatcttgacttg

SEQ ID NO: 1419 - DNA, 33 bp, Artificial; identical to SEQ ID NO: 979
  Humanized Antibody

SEQ ID NO: 1420 - DNA, 990 bp, Artificial; identical to SEQ ID NO: 460
  Humanized Antibody

SEQ ID NO: 1421 - protein, 214 aa, Artificial
  Humanized Antibody
QLTQSPSTLSASVGDRVTITCQSSESVYGNYLAWFQQKPGKAPKFLIYEASKLESGVPSRFSGSGSGTEFTLTISSLQPDDFATYYCAGGDISEGVAFGGGTKVEIKRTVAAPSVFIFPPSDEQLKSGTASVVCLLNNFYPREAKVQWKVDNALQSGNSQESVTEQDSKDSTYSLSSTLTLSKADYEKHKVYACEVTHQGLSSPVTKSFNRGEC

SEQ ID NO: 1422 - protein, 108 aa, Artificial
  Humanized Antibody
QLTQSPSTLSASVGDRVTITCQSSESVYGNYLAWFQQKPGKAPKFLIYEASKLESGVPSRFSGSGSGTEFTLTISSLQPDDFATYYCAGGDISEGVAFGGGTKVEIKR

SEQ ID NO: 1423 - protein, 21 aa, Artificial
  Humanized Antibody
QLTQSPSTLSASVGDRVTITC

SEQ ID NO: 1424 - protein, 12 aa, Oryctolagus cuniculus
QSSESVYGNYLA

SEQ ID NO: 1425 - protein, 15 aa, Artificial
  Humanized Antibody
WFQQKPGKAPKFLIY

SEQ ID NO: 1426 - protein, 7 aa, Oryctolagus cuniculus
EASKLES

SEQ ID NO: 1427 - protein, 32 aa, Artificial; identical to SEQ ID NO: 987
  Humanized Antibody

SEQ ID NO: 1428 - protein, 10 aa, Oryctolagus cuniculus
AGGDISEGVA

SEQ ID NO: 1429 - protein, 11 aa, Artificial
  Humanized Antibody
FGGGTKVEIKR

SEQ ID NO: 1430 - protein, 106 aa, Artificial; identical to SEQ ID NO: 430
  Humanized Antibody

SEQ ID NO: 1431 - DNA, 642 bp, Artificial
  Humanized Antibody
cagctgacccagtctccttccaccctgtctgcatctgtaggagacagagtcaccatcacttgtcagtccagtgagagtgtttacggtaactacttagcctggtttcagcagaaaccaggaaaagcccctaagttcctgatctatgaagcatccaaactggaatctggagtcccatcaaggttcagcggcagtggatctggaacagaattcactctcaccatcagcagcctgcagcctgatgattttgcaacttactactgtgcaggcggtgatattagtgaaggtgttgctttcggcggaggaaccaaggtggaaatcaaacgtacggtagcggccccatctgtcttcatcttcccgccatctgatgagcagttgaaatctggaactgcctctgttgtgtgcctgctgaataacttctatcccagagaggccaaagtacagtggaaggtggataacgccctccaatcgggtaactcccaggagagtgtcacagagcaggacagcaaggacagcacctacagcctcagcagcaccctgacgctgagcaaagcagactacgagaaacacaaagtctacgcctgcgaagtcacccatcagggcctgagctcgcccgtcacaaagagcttcaacaggggagagtgt

SEQ ID NO: 1432 - DNA, 324 bp, Artificial
  Humanized Antibody
cagctgacccagtctccttccaccctgtctgcatctgtaggagacagagtcaccatcacttgtcagtccagtgagagtgtttacggtaactacttagcctggtttcagcagaaaccaggaaaagcccctaagttcctgatctatgaagcatccaaactggaatctggagtcccatcaaggttcagcggcagtggatctggaacagaattcactctcaccatcagcagcctgcagcctgatgattttgcaacttactactgtgcaggcggtgatattagtgaaggtgttgctttcggcggaggaaccaaggtggaaatcaaacgt

SEQ ID NO: 1433 - DNA, 63 bp, Artificial
  Humanized Antibody
cagctgacccagtctccttccaccctgtctgcatctgtaggagacagagtcaccatcacttgt

SEQ ID NO: 1434 - DNA, 36 bp, Oryctolagus cuniculus; identical to SEQ ID NO: 434

SEQ ID NO: 1435 - DNA, 45 bp, Artificial; identical to SEQ ID NO: 995
  Humanized Antibody

SEQ ID NO: 1436 - DNA, 21 bp, Oryctolagus cuniculus
gaagcatccaaactggaatct

SEQ ID NO: 1437 - DNA, 96 bp, Artificial; identical to SEQ ID NO: 997
  Humanized Antibody

SEQ ID NO: 1438 - DNA, 30 bp, Oryctolagus cuniculus; identical to SEQ ID NO: 438

SEQ ID NO: 1439 - DNA, 33 bp, Artificial; identical to SEQ ID NO: 999
  Humanized Antibody

SEQ ID NO: 1440 - DNA, 318 bp, Artificial; identical to SEQ ID NO: 440
  Humanized Antibody

SEQ ID NO: 1441 - protein, 442 aa, Artificial; identical to SEQ ID NO: 961
  Humanized Antibody

SEQ ID NO: 1442 - protein, 112 aa, Artificial; identical to SEQ ID NO: 962
  Humanized Antibody

SEQ ID NO: 1443 - protein, 30 aa, Artificial; identical to SEQ ID NO: 963
  Humanized Antibody

SEQ ID NO: 1444 - protein, 5 aa, Oryctolagus cuniculus
SYYMT

SEQ ID NO: 1445 - protein, 14 aa, Artificial
  Humanized Antibody
WVRQAPGKGLEWIG

SEQ ID NO: 1446 - protein, 16 aa, Oryctolagus cuniculus
FIDAGGDAYYASWAKG

SEQ ID NO: 1447 - protein, 32 aa, Artificial; identical to SEQ ID NO: 967
  Humanized Antibody

SEQ ID NO: 1448 - protein, 4 aa, Oryctolagus cuniculus
DLDL

SEQ ID NO: 1449 - protein, 11 aa, Artificial
  Humanized Antibody
WGQGTLVTVSS

SEQ ID NO: 1450 - protein, 330 aa, Artificial; identical to SEQ ID NO: 450
  Humanized Antibody

SEQ ID NO: 1451 - DNA, 1326 bp, Artificial; identical to SEQ ID NO: 971
  Humanized Antibody

SEQ ID NO: 1452 - DNA, 336 bp, Artificial; identical to SEQ ID NO: 972
  Humanized Antibody

SEQ ID NO: 1453 - DNA, 90 bp, Artificial; identical to SEQ ID NO: 973
  Humanized Antibody

SEQ ID NO: 1454 - DNA, 15 bp, Oryctolagus cuniculus
agctactacatgacc

SEQ ID NO: 1455 - DNA, 42 bp, Artificial; identical to SEQ ID NO: 975
  Humanized Antibody

SEQ ID NO: 1456 - DNA, 48 bp, Oryctolagus cuniculus; identical to SEQ ID NO: 416

SEQ ID NO: 1457 - DNA, 96 bp, Artificial; identical to SEQ ID NO: 977
  Humanized Antibody

SEQ ID NO: 1458 - DNA, 12 bp, Oryctolagus cuniculus
gatcttgacttg

SEQ ID NO: 1459 - DNA, 33 bp, Artificial; identical to SEQ ID NO: 979
  Humanized Antibody

SEQ ID NO: 1460 - DNA, 990 bp, Artificial; identical to SEQ ID NO: 460
  Humanized Antibody

SEQ ID NO: 1461 - protein, 215 aa, Artificial
  Humanized Antibody
QVLTQSPSTLSASVGDRVTITCQSSESVYGNYLAWFQQKPGKAPKFLIYEASKLESGVPSRFSGSGSGTEFTLTISSLQPDDFATYYCAGGDISEGVAFGGGTKVEIKRTVAAPSVFIFPPSDEQLKSGTASVVCLLNNFYPREAKVQWKVDNALQSGNSQESVTEQDSKDSTYSLSSTLTLSKADYEKHKVYACEVTHQGLSSPVTKSFNRGEC

SEQ ID NO: 1462 - protein, 109 aa, Artificial
  Humanized Antibody
QVLTQSPSTLSASVGDRVTITCQSSESVYGNYLAWFQQKPGKAPKFLIYEASKLESGVPSRFSGSGSGTEFTLTISSLQPDDFATYYCAGGDISEGVAFGGGTKVEIKR

SEQ ID NO: 1463 - protein, 22 aa, Artificial
  Humanized Antibody
QVLTQSPSTLSASVGDRVTITC

SEQ ID NO: 1464 - protein, 12 aa, Oryctolagus cuniculus
QSSESVYGNYLA

SEQ ID NO: 1465 - protein, 15 aa, Artificial
  Humanized Antibody
WFQQKPGKAPKFLIY

SEQ ID NO: 1466 - protein, 7 aa, Oryctolagus cuniculus
EASKLES

SEQ ID NO: 1467 - protein, 32 aa, Artificial; identical to SEQ ID NO: 987
  Humanized Antibody

SEQ ID NO: 1468 - protein, 10 aa, Oryctolagus cuniculus
AGGDISEGVA

SEQ ID NO: 1469 - protein, 11 aa, Artificial
  Humanized Antibody
FGGGTKVEIKR

SEQ ID NO: 1470 - protein, 106 aa, Artificial; identical to SEQ ID NO: 430
  Humanized Antibody

SEQ ID NO: 1471 - DNA, 645 bp, Artificial
  Humanized Antibody
caggtgctgacccagtctccttccaccctgtctgcatctgtaggagacagagtcaccatcacttgtcagtccagtgagagtgtttacggtaactacttagcctggtttcagcagaaaccaggaaaagcccctaagttcctgatctatgaagcatccaaactggaatctggagtcccatcaaggttcagcggcagtggatctggaacagaattcactctcaccatcagcagcctgcagcctgatgattttgcaacttactactgtgcaggcggtgatattagtgaaggtgttgctttcggcggaggaaccaaggtggaaatcaaacgtacggtagcggccccatctgtcttcatcttcccgccatctgatgagcagttgaaatctggaactgcctctgttgtgtgcctgctgaataacttctatcccagagaggccaaagtacagtggaaggtggataacgccctccaatcgggtaactcccaggagagtgtcacagagcaggacagcaaggacagcacctacagcctcagcagcaccctgacgctgagcaaagcagactacgagaaacacaaagtctacgcctgcgaagtcacccatcagggcctgagctcgcccgtcacaaagagcttcaacaggggagagtgt

SEQ ID NO: 1472 - DNA, 327 bp, Artificial
  Humanized Antibody
caggtgctgacccagtctccttccaccctgtctgcatctgtaggagacagagtcaccatcacttgtcagtccagtgagagtgtttacggtaactacttagcctggtttcagcagaaaccaggaaaagcccctaagttcctgatctatgaagcatccaaactggaatctggagtcccatcaaggttcagcggcagtggatctggaacagaattcactctcaccatcagcagcctgcagcctgatgattttgcaacttactactgtgcaggcggtgatattagtgaaggtgttgctttcggcggaggaaccaaggtggaaatcaaacgt

SEQ ID NO: 1473 - DNA, 66 bp, Artificial
  Humanized Antibody
caggtgctgacccagtctccttccaccctgtctgcatctgtaggagacagagtcaccatcacttgt

SEQ ID NO: 1474 - DNA, 36 bp, Oryctolagus cuniculus; identical to SEQ ID NO: 434

SEQ ID NO: 1475 - DNA, 45 bp, Artificial; identical to SEQ ID NO: 995
  Humanized Antibody

SEQ ID NO: 1476 - DNA, 21 bp, Oryctolagus cuniculus
gaagcatccaaactggaatct

SEQ ID NO: 1477 - DNA, 96 bp, Artificial; identical to SEQ ID NO: 997
  Humanized Antibody

SEQ ID NO: 1478 - DNA, 30 bp, Oryctolagus cuniculus; identical to SEQ ID NO: 438

SEQ ID NO: 1479 - DNA, 33 bp, Artificial; identical to SEQ ID NO: 999
  Humanized Antibody

SEQ ID NO: 1480 - DNA, 318 bp, Artificial; identical to SEQ ID NO: 440
  Humanized Antibody

SEQ ID NO: 1481 - protein, 442 aa, Artificial; identical to SEQ ID NO: 1201
  Humanized Antibody

SEQ ID NO: 1482 - protein, 112 aa, Artificial; identical to SEQ ID NO: 1202
  Humanized Antibody

SEQ ID NO: 1483 - protein, 30 aa, Artificial; identical to SEQ ID NO: 1203
  Humanized Antibody

SEQ ID NO: 1484 - protein, 5 aa, Oryctolagus cuniculus
SYYMT

SEQ ID NO: 1485 - protein, 14 aa, Artificial
  Humanized Antibody
WVRQAPGKGLEWIG

SEQ ID NO: 1486 - protein, 16 aa, Oryctolagus cuniculus
FIDAGGSAYYATWAKG

SEQ ID NO: 1487 - protein, 32 aa, Artificial; identical to SEQ ID NO: 967
  Humanized Antibody

SEQ ID NO: 1488 - protein, 4 aa, Oryctolagus cuniculus
DLDL

SEQ ID NO: 1489 - protein, 11 aa, Artificial
  Humanized Antibody
WGQGTLVTVSS

SEQ ID NO: 1490 - protein, 330 aa, Artificial; identical to SEQ ID NO: 450
  Humanized Antibody

SEQ ID NO: 1491 - DNA, 1326 bp, Artificial; identical to SEQ ID NO: 1211
  Humanized Antibody

SEQ ID NO: 1492 - DNA, 336 bp, Artificial; identical to SEQ ID NO: 1212
  Humanized Antibody

SEQ ID NO: 1493 - DNA, 90 bp, Artificial; identical to SEQ ID NO: 1213
  Humanized Antibody

SEQ ID NO: 1494 - DNA, 15 bp, Oryctolagus cuniculus
agctactacatgacc

SEQ ID NO: 1495 - DNA, 42 bp, Artificial; identical to SEQ ID NO: 975
  Humanized Antibody

SEQ ID NO: 1496 - DNA, 48 bp, Oryctolagus cuniculus; identical to SEQ ID NO: 856

SEQ ID NO: 1497 - DNA, 96 bp, Artificial; identical to SEQ ID NO: 977
  Humanized Antibody

SEQ ID NO: 1498 - DNA, 12 bp, Oryctolagus cuniculus
gatcttgacttg

SEQ ID NO: 1499 - DNA, 33 bp, Artificial; identical to SEQ ID NO: 979
  Humanized Antibody

SEQ ID NO: 1500 - DNA, 990 bp, Artificial; identical to SEQ ID NO: 460
  Humanized Antibody

SEQ ID NO: 1501 - protein, 215 aa, Artificial
  Humanized Antibody
AVLTQSPSTLSASVGDRVTITCKSSESVYGDYLAWFQQKPGKAPKQLIYDASTLASGVPSRFSGSGSGTEFTLTISSLQPDDFATYYCAGGYVSAGVAFGGGTKVEIKRTVAAPSVFIFPPSDEQLKSGTASVVCLLNNFYPREAKVQWKVDNALQSGNSQESVTEQDSKDSTYSLSSTLTLSKADYEKHKVYACEVTHQGLSSPVTKSFNRGEC

SEQ ID NO: 1502 - protein, 109 aa, Artificial
  Humanized Antibody
AVLTQSPSTLSASVGDRVTITCKSSESVYGDYLAWFQQKPGKAPKQLIYDASTLASGVPSRFSGSGSGTEFTLTISSLQPDDFATYYCAGGYVSAGVAFGGGTKVEIKR

SEQ ID NO: 1503 - protein, 22 aa, Artificial
  Humanized Antibody
AVLTQSPSTLSASVGDRVTITC

SEQ ID NO: 1504 - protein, 12 aa, Oryctolagus cuniculus
KSSESVYGDYLA

SEQ ID NO: 1505 - protein, 15 aa, Artificial
  Humanized Antibody
WFQQKPGKAPKQLIY

SEQ ID NO: 1506 - protein, 7 aa, Oryctolagus cuniculus
DASTLAS

SEQ ID NO: 1507 - protein, 32 aa, Artificial; identical to SEQ ID NO: 987
  Humanized Antibody

SEQ ID NO: 1508 - protein, 10 aa, Oryctolagus cuniculus
AGGYVSAGVA

SEQ ID NO: 1509 - protein, 11 aa, Artificial
  Humanized Antibody
FGGGTKVEIKR

SEQ ID NO: 1510 - protein, 106 aa, Artificial; identical to SEQ ID NO: 430
  Humanized Antibody

SEQ ID NO: 1511 - DNA, 645 bp, Artificial
  Humanized Antibody
gccgtgctgacccagtctccttccaccctgtctgcatctgtaggagacagagtcaccatcacttgtaagtccagtgagagcgtttatggtgactacttagcctggtttcagcagaaaccaggaaaagcccctaagcaactgatctatgatgcatccactctggcatctggagtcccatcaaggttcagcggcagtggatctggaacagaattcactctcaccatcagcagcctgcagcctgatgattttgcaacttactactgtgcaggcggttatgttagtgcaggtgttgctttcggcggaggaaccaaggtggaaatcaaacgtacggtagcggccccatctgtcttcatcttcccgccatctgatgagcagttgaaatctggaactgcctctgttgtgtgcctgctgaataacttctatcccagagaggccaaagtacagtggaaggtggataacgccctccaatcgggtaactcccaggagagtgtcacagagcaggacagcaaggacagcacctacagcctcagcagcaccctgacgctgagcaaagcagactacgagaaacacaaagtctacgcctgcgaagtcacccatcagggcctgagctcgcccgtcacaaagagcttcaacaggggagagtgt

SEQ ID NO: 1512 - DNA, 327 bp, Artificial
  Humanized Antibody
gccgtgctgacccagtctccttccaccctgtctgcatctgtaggagacagagtcaccatcacttgtaagtccagtgagagcgtttatggtgactacttagcctggtttcagcagaaaccaggaaaagcccctaagcaactgatctatgatgcatccactctggcatctggagtcccatcaaggttcagcggcagtggatctggaacagaattcactctcaccatcagcagcctgcagcctgatgattttgcaacttactactgtgcaggcggttatgttagtgcaggtgttgctttcggcggaggaaccaaggtggaaatcaaacgt

SEQ ID NO: 1513 - DNA, 66 bp, Artificial; identical to SEQ ID NO: 1313
  Humanized Antibody

SEQ ID NO: 1514 - DNA, 36 bp, Oryctolagus cuniculus; identical to SEQ ID NO: 874

SEQ ID NO: 1515 - DNA, 45 bp, Artificial; identical to SEQ ID NO: 1235
  Humanized Antibody

SEQ ID NO: 1516 - DNA, 21 bp, Oryctolagus cuniculus
gatgcatccactctggcatct

SEQ ID NO: 1517 - DNA, 96 bp, Artificial; identical to SEQ ID NO: 997
  Humanized Antibody

SEQ ID NO: 1518 - DNA, 30 bp, Oryctolagus cuniculus; identical to SEQ ID NO: 878

SEQ ID NO: 1519 - DNA, 33 bp, Artificial; identical to SEQ ID NO: 999
  Humanized Antibody

SEQ ID NO: 1520 - DNA, 318 bp, Artificial; identical to SEQ ID NO: 440
  Humanized Antibody

SEQ ID NO: 1521 - protein, 442 aa, Artificial; identical to SEQ ID NO: 1201
  Humanized Antibody

SEQ ID NO: 1522 - protein, 112 aa, Artificial; identical to SEQ ID NO: 1202
  Humanized Antibody

SEQ ID NO: 1523 - protein, 30 aa, Artificial; identical to SEQ ID NO: 1203
  Humanized Antibody

SEQ ID NO: 1524 - protein, 5 aa, Oryctolagus cuniculus
SYYMT

SEQ ID NO: 1525 - protein, 14 aa, Artificial
  Humanized Antibody
WVRQAPGKGLEWIG

SEQ ID NO: 1526 - protein, 16 aa, Oryctolagus cuniculus
FIDAGGSAYYATWAKG

SEQ ID NO: 1527 - protein, 32 aa, Artificial; identical to SEQ ID NO: 967
  Humanized Antibody

SEQ ID NO: 1528 - protein, 4 aa, Oryctolagus cuniculus
DLDL

SEQ ID NO: 1529 - protein, 11 aa, Artificial
  Humanized Antibody
WGQGTLVTVSS

SEQ ID NO: 1530 - protein, 330 aa, Artificial; identical to SEQ ID NO: 450
  Humanized Antibody

SEQ ID NO: 1531 - DNA, 1326 bp, Artificial; identical to SEQ ID NO: 1211
  Humanized Antibody

SEQ ID NO: 1532 - DNA, 336 bp, Artificial; identical to SEQ ID NO: 1212
  Humanized Antibody

SEQ ID NO: 1533 - DNA, 90 bp, Artificial; identical to SEQ ID NO: 1213
  Humanized Antibody

SEQ ID NO: 1534 - DNA, 15 bp, Oryctolagus cuniculus
agctactacatgacc

SEQ ID NO: 1535 - DNA, 42 bp, Artificial; identical to SEQ ID NO: 975
  Humanized Antibody

SEQ ID NO: 1536 - DNA, 48 bp, Oryctolagus cuniculus; identical to SEQ ID NO: 856

SEQ ID NO: 1537 - DNA, 96 bp, Artificial; identical to SEQ ID NO: 977
  Humanized Antibody

SEQ ID NO: 1538 - DNA, 12 bp, Oryctolagus cuniculus
gatcttgacttg

SEQ ID NO: 1539 - DNA, 33 bp, Artificial; identical to SEQ ID NO: 979
  Humanized Antibody

SEQ ID NO: 1540 - DNA, 990 bp, Artificial; identical to SEQ ID NO: 460
  Humanized Antibody

SEQ ID NO: 1541 - protein, 216 aa, Artificial
  Humanized Antibody
DIQLTQSPSTLSASVGDRVTITCKSSESVYGDYLAWFQQKPGKAPKQLIYDASTLASGVPSRFSGSGSGTEFTLTISSLQPDDFATYYCAGGYVSAGVAFGGGTKVEIKRTVAAPSVFIFPPSDEQLKSGTASVVCLLNNFYPREAKVQWKVDNALQSGNSQESVTEQDSKDSTYSLSSTLTLSKADYEKHKVYACEVTHQGLSSPVTKSFNRGEC

SEQ ID NO: 1542 - protein, 110 aa, Artificial
  Humanized Antibody
DIQLTQSPSTLSASVGDRVTITCKSSESVYGDYLAWFQQKPGKAPKQLIYDASTLASGVPSRFSGSGSGTEFTLTISSLQPDDFATYYCAGGYVSAGVAFGGGTKVEIKR

SEQ ID NO: 1543 - protein, 23 aa, Artificial
  Humanized Antibody
DIQLTQSPSTLSASVGDRVTITC

SEQ ID NO: 1544 - protein, 12 aa, Oryctolagus cuniculus
KSSESVYGDYLA

SEQ ID NO: 1545 - protein, 15 aa, Artificial
  Humanized Antibody
WFQQKPGKAPKQLIY

SEQ ID NO: 1546 - protein, 7 aa, Oryctolagus cuniculus
DASTLAS

SEQ ID NO: 1547 - protein, 32 aa, Artificial; identical to SEQ ID NO: 987
  Humanized Antibody

SEQ ID NO: 1548 - protein, 10 aa, Oryctolagus cuniculus
AGGYVSAGVA

SEQ ID NO: 1549 - protein, 11 aa, Artificial
  Humanized Antibody
FGGGTKVEIKR

SEQ ID NO: 1550 - protein, 106 aa, Artificial; identical to SEQ ID NO: 430
  Humanized Antibody

SEQ ID NO: 1551 - DNA, 648 bp, Artificial
  Humanized Antibody
gacatccagctgacccagtctccttccaccctgtctgcatctgtaggagacagagtcaccatcacttgtaagtccagtgagagcgtttatggtgactacttagcctggtttcagcagaaaccaggaaaagcccctaagcaactgatctatgatgcatccactctggcatctggagtcccatcaaggttcagcggcagtggatctggaacagaattcactctcaccatcagcagcctgcagcctgatgattttgcaacttactactgtgcaggcggttatgttagtgcaggtgttgctttcggcggaggaaccaaggtggaaatcaaacgtacggtagcggccccatctgtcttcatcttcccgccatctgatgagcagttgaaatctggaactgcctctgttgtgtgcctgctgaataacttctatcccagagaggccaaagtacagtggaaggtggataacgccctccaatcgggtaactcccaggagagtgtcacagagcaggacagcaaggacagcacctacagcctcagcagcaccctgacgctgagcaaagcagactacgagaaacacaaagtctacgcctgcgaagtcacccatcagggcctgagctcgcccgtcacaaagagcttcaacaggggagagtgt

SEQ ID NO: 1552 - DNA, 330 bp, Artificial
  Humanized Antibody
gacatccagctgacccagtctccttccaccctgtctgcatctgtaggagacagagtcaccatcacttgtaagtccagtgagagcgtttatggtgactacttagcctggtttcagcagaaaccaggaaaagcccctaagcaactgatctatgatgcatccactctggcatctggagtcccatcaaggttcagcggcagtggatctggaacagaattcactctcaccatcagcagcctgcagcctgatgattttgcaacttactactgtgcaggcggttatgttagtgcaggtgttgctttcggcggaggaaccaaggtggaaatcaaacgt

SEQ ID NO: 1553 - DNA, 69 bp, Artificial; identical to SEQ ID NO: 1353
  Humanized Antibody

SEQ ID NO: 1554 - DNA, 36 bp, Oryctolagus cuniculus; identical to SEQ ID NO: 874

SEQ ID NO: 1555 - DNA, 45 bp, Artificial; identical to SEQ ID NO: 1235
  Humanized Antibody

SEQ ID NO: 1556 - DNA, 21 bp, Oryctolagus cuniculus
gatgcatccactctggcatct

SEQ ID NO: 1557 - DNA, 96 bp, Artificial; identical to SEQ ID NO: 997
  Humanized Antibody

SEQ ID NO: 1558 - DNA, 30 bp, Oryctolagus cuniculus; identical to SEQ ID NO: 878

SEQ ID NO: 1559 - DNA, 33 bp, Artificial; identical to SEQ ID NO: 999
  Humanized Antibody

SEQ ID NO: 1560 - DNA, 318 bp, Artificial; identical to SEQ ID NO: 440
  Humanized Antibody

SEQ ID NO: 1561 - protein, 442 aa, Artificial; identical to SEQ ID NO: 1201
  Humanized Antibody

SEQ ID NO: 1562 - protein, 112 aa, Artificial; identical to SEQ ID NO: 1202
  Humanized Antibody

SEQ ID NO: 1563 - protein, 30 aa, Artificial; identical to SEQ ID NO: 1203
  Humanized Antibody

SEQ ID NO: 1564 - protein, 5 aa, Oryctolagus cuniculus
SYYMT

SEQ ID NO: 1565 - protein, 14 aa, Artificial
  Humanized Antibody
WVRQAPGKGLEWIG

SEQ ID NO: 1566 - protein, 16 aa, Oryctolagus cuniculus
FIDAGGSAYYATWAKG

SEQ ID NO: 1567 - protein, 32 aa, Artificial; identical to SEQ ID NO: 967
  Humanized Antibody

SEQ ID NO: 1568 - protein, 4 aa, Oryctolagus cuniculus
DLDL

SEQ ID NO: 1569 - protein, 11 aa, Artificial
  Humanized Antibody
WGQGTLVTVSS

SEQ ID NO: 1570 - protein, 330 aa, Artificial; identical to SEQ ID NO: 450
  Humanized Antibody

SEQ ID NO: 1571 - DNA, 1326 bp, Artificial; identical to SEQ ID NO: 1211
  Humanized Antibody

SEQ ID NO: 1572 - DNA, 336 bp, Artificial; identical to SEQ ID NO: 1212
  Humanized Antibody

SEQ ID NO: 1573 - DNA, 90 bp, Artificial; identical to SEQ ID NO: 1213
  Humanized Antibody

SEQ ID NO: 1574 - DNA, 15 bp, Oryctolagus cuniculus
agctactacatgacc

SEQ ID NO: 1575 - DNA, 42 bp, Artificial; identical to SEQ ID NO: 975
  Humanized Antibody

SEQ ID NO: 1576 - DNA, 48 bp, Oryctolagus cuniculus; identical to SEQ ID NO: 856

SEQ ID NO: 1577 - DNA, 96 bp, Artificial; identical to SEQ ID NO: 977
  Humanized Antibody

SEQ ID NO: 1578 - DNA, 12 bp, Oryctolagus cuniculus
gatcttgacttg

SEQ ID NO: 1579 - DNA, 33 bp, Artificial; identical to SEQ ID NO: 979
  Humanized Antibody

SEQ ID NO: 1580 - DNA, 990 bp, Artificial; identical to SEQ ID NO: 460
  Humanized Antibody

SEQ ID NO: 1581 - protein, 216 aa, Artificial
  Humanized Antibody
DIVLTQSPSTLSASVGDRVTITCKSSESVYGDYLAWFQQKPGKAPKQLIYDASTLASGVPSRFSGSGSGTEFTLTISSLQPDDFATYYCAGGYVSAGVAFGGGTKVEIKRTVAAPSVFIFPPSDEQLKSGTASVVCLLNNFYPREAKVQWKVDNALQSGNSQESVTEQDSKDSTYSLSSTLTLSKADYEKHKVYACEVTHQGLSSPVTKSFNRGEC

SEQ ID NO: 1582 - protein, 110 aa, Artificial
  Humanized Antibody
DIVLTQSPSTLSASVGDRVTITCKSSESVYGDYLAWFQQKPGKAPKQLIYDASTLASGVPSRFSGSGSGTEFTLTISSLQPDDFATYYCAGGYVSAGVAFGGGTKVEIKR

SEQ ID NO: 1583 - protein, 23 aa, Artificial
  Humanized Antibody
DIVLTQSPSTLSASVGDRVTITC

SEQ ID NO: 1584 - protein, 12 aa, Oryctolagus cuniculus
KSSESVYGDYLA

SEQ ID NO: 1585 - protein, 15 aa, Artificial
  Humanized Antibody
WFQQKPGKAPKQLIY

SEQ ID NO: 1586 - protein, 7 aa, Oryctolagus cuniculus
DASTLAS

SEQ ID NO: 1587 - protein, 32 aa, Artificial; identical to SEQ ID NO: 987
  Humanized Antibody

SEQ ID NO: 1588 - protein, 10 aa, Oryctolagus cuniculus
AGGYVSAGVA

SEQ ID NO: 1589 - protein, 11 aa, Artificial
  Humanized Antibody
FGGGTKVEIKR

SEQ ID NO: 1590 - protein, 106 aa, Artificial; identical to SEQ ID NO: 430
  Humanized Antibody

SEQ ID NO: 1591 - DNA, 648 bp, Artificial
  Humanized Antibody
gacatcgtgctgacccagtctccttccaccctgtctgcatctgtaggagacagagtcaccatcacttgtaagtccagtgagagcgtttatggtgactacttagcctggtttcagcagaaaccaggaaaagcccctaagcaactgatctatgatgcatccactctggcatctggagtcccatcaaggttcagcggcagtggatctggaacagaattcactctcaccatcagcagcctgcagcctgatgattttgcaacttactactgtgcaggcggttatgttagtgcaggtgttgctttcggcggaggaaccaaggtggaaatcaaacgtacggtagcggccccatctgtcttcatcttcccgccatctgatgagcagttgaaatctggaactgcctctgttgtgtgcctgctgaataacttctatcccagagaggccaaagtacagtggaaggtggataacgccctccaatcgggtaactcccaggagagtgtcacagagcaggacagcaaggacagcacctacagcctcagcagcaccctgacgctgagcaaagcagactacgagaaacacaaagtctacgcctgcgaagtcacccatcagggcctgagctcgcccgtcacaaagagcttcaacaggggagagtgt

SEQ ID NO: 1592 - DNA, 330 bp, Artificial
  Humanized Antibody
gacatcgtgctgacccagtctccttccaccctgtctgcatctgtaggagacagagtcaccatcacttgtaagtccagtgagagcgtttatggtgactacttagcctggtttcagcagaaaccaggaaaagcccctaagcaactgatctatgatgcatccactctggcatctggagtcccatcaaggttcagcggcagtggatctggaacagaattcactctcaccatcagcagcctgcagcctgatgattttgcaacttactactgtgcaggcggttatgttagtgcaggtgttgctttcggcggaggaaccaaggtggaaatcaaacgt

SEQ ID NO: 1593 - DNA, 69 bp, Artificial; identical to SEQ ID NO: 1393
  Humanized Antibody

SEQ ID NO: 1594 - DNA, 36 bp, Oryctolagus cuniculus; identical to SEQ ID NO: 874

SEQ ID NO: 1595 - DNA, 45 bp, Artificial; identical to SEQ ID NO: 1235
  Humanized Antibody

SEQ ID NO: 1596 - DNA, 21 bp, Oryctolagus cuniculus
gatgcatccactctggcatct

SEQ ID NO: 1597 - DNA, 96 bp, Artificial; identical to SEQ ID NO: 997
  Humanized Antibody

SEQ ID NO: 1598 - DNA, 30 bp, Oryctolagus cuniculus; identical to SEQ ID NO: 878

SEQ ID NO: 1599 - DNA, 33 bp, Artificial; identical to SEQ ID NO: 999
  Humanized Antibody

SEQ ID NO: 1600 - DNA, 318 bp, Artificial; identical to SEQ ID NO: 440
  Humanized Antibody